European Patent Specification EP 3 873 512 B1, published January 14, 2026. Title: EpCAM antibodies, activatable antibodies, and immunoconjugates, and uses thereof. Applicant: ImmunoGen, Inc., CytomX Therapeutics, Inc. The sequence listing filed with the application follows.

SEQUENCE LISTING (317 sequences)

SEQ ID NO: 1 - protein, 242 aa, Artificial Sequence
  Synthetic Polypeptide
QEECVCENYKLAVNCFVNNNRQCQCTSVGAQNTVICSKLAAKCLVMKAEMNGSKLGRRAKPEGALQNNDGLYDPDCDESGLFKAKQCNGTSMCWCVNTAGVRRTDKDTEITCSERVRTYWIIIELKHKAREKPYDSKSLRTALQKEITTRYQLDPKFITSILYENNVITIDLVQNSSQKTQNDVDIADVAYYFEKDVKGESLFHSKKMDLTVNGEQLDLDPGQTLIYYVDEKAPEFSMQGLK

SEQ ID NO: 2 - protein, 36 aa, Artificial Sequence
  Synthetic Polypeptide
QEECVCENYKLAVNCFVNNNRQCQCTSVGAQNTVIC

SEQ ID NO: 3 - protein, 70 aa, Artificial Sequence
  Synthetic Polypeptide
CLVMKAEMNGSKLGRRAKPEGALQNNDGLYDPDCDESGLFKAKQCNGTSMCWCVNTAGVRRTDKDTEITC

SEQ ID NO: 4 - protein, 130 aa, Artificial Sequence
  Synthetic Polypeptide
SERVRTYWIIIELKHKAREKPYDSKSLRTALQKEITTRYQLDPKFITSILYENNVITIDLVQNSSQKTQNDVDIADVAYYFEKDVKGESLFHSKKMDLTVNGEQLDLDPGQTLIYYVDEKAPEFSMQGLK

SEQ ID NO: 5 - protein, 5 aa, Artificial Sequence
  Synthetic Polypeptide
  MISC_FEATURE (1)..(1): Xaa is any amino acid
  MISC_FEATURE (3)..(3): Xaa is Y,N,F,S,H,D,L,I,W
  MISC_FEATURE (4)..(4): Xaa is I or M
XYXXH

SEQ ID NO: 6 - protein, 5 aa, Artificial Sequence
  Synthetic Polypeptide
  MISC_FEATURE (3)..(3): Xaa is Y,N,F,S,H,D,L,I,W
  MISC_FEATURE (3)..(3): Xaa is Y,N,F,S,H,D,L,I, or W
NYXIH

SEQ ID NO: 7 - protein, 17 aa, Artificial Sequence
  Synthetic Polypeptide
  MISC_FEATURE (2)..(2): Xaa is I, S, or V
  MISC_FEATURE (3)..(3): Xaa is Y or N
  MISC_FEATURE (6)..(6): Xaa is N or D
  MISC_FEATURE (12)..(12): Xaa is N or S
  MISC_FEATURE (13)..(13): Xaa is E or Q
  MISC_FEATURE (17)..(17): Xaa is K or Q
WXXPGXVYIQYXXKFKX

SEQ ID NO: 8 - protein, 7 aa, Artificial Sequence
  Synthetic Polypeptide
  MISC_FEATURE (1)..(1): Xaa is D or E
  MISC_FEATURE (3)..(3): Xaa is P,A,S,Y,F,G,T,V, or A
  MISC_FEATURE (4)..(4): Xaa is Y or w
  MISC_FEATURE (4)..(4): Xaa is Y or W
XGXXFAY

SEQ ID NO: 9 - protein, 7 aa, Artificial Sequence
  Synthetic Polypeptide
  MISC_FEATURE (4)..(4): Xaa is Y or W
DGPXFAY

SEQ ID NO: 10 - protein, 16 aa, Artificial Sequence
  Synthetic Polypeptide
  MISC_FEATURE (10)..(10): Xaa is N or D
  MISC_FEATURE (12)..(12): Xaa is F or I
  MISC_FEATURE (16)..(16): Xaa is Y or S
RSSRSLLHSXGXTYLX

SEQ ID NO: 11 - protein, 9 aa, Artificial Sequence
  Synthetic Polypeptide
  MISC_FEATURE (1)..(1): Xaa is A,K, or Q
  MISC_FEATURE (1)..(1): Xaa is A,L, or Q
  MISC_FEATURE (3)..(3): Xaa is S,G,Y,or N
  MISC_FEATURE (8)..(8): Xaa is N or W
XQXLELPXT

SEQ ID NO: 12 - protein, 9 aa, Artificial Sequence
  Synthetic Polypeptide
  MISC_FEATURE (3)..(3): Xaa is S, G, Y, or N
AQXLELPNT

SEQ ID NO: 13 - protein, 5 aa, Artificial Sequence
  Synthetic Polypeptide
NYYIH

SEQ ID NO: 14 - protein, 17 aa, Artificial Sequence
  Synthetic Polypeptide
WIYPGNVYIQYNEKFKG

SEQ ID NO: 15 - protein, 7 aa, Artificial Sequence
  Synthetic Polypeptide
DGPWFAY

SEQ ID NO: 16 - protein, 5 aa, Artificial Sequence
  Synthetic Polypeptide
SYYIH

SEQ ID NO: 17 - protein, 5 aa, Artificial Sequence
  Synthetic Polypeptide
NYNIH

SEQ ID NO: 18 - protein, 5 aa, Artificial Sequence
  Synthetic Polypeptide
NYFIH

SEQ ID NO: 19 - protein, 5 aa, Artificial Sequence
  Synthetic Polypeptide
NYSIH

SEQ ID NO: 20 - protein, 5 aa, Artificial Sequence
  Synthetic Polypeptide
NYWIH

SEQ ID NO: 21 - protein, 5 aa, Artificial Sequence
  Synthetic Polypeptide
NYYMH

SEQ ID NO: 22 - protein, 5 aa, Artificial Sequence
  Synthetic Polypeptide
NYHIH

SEQ ID NO: 23 - protein, 5 aa, Artificial Sequence
  Synthetic Polypeptide
NYDIH

SEQ ID NO: 24 - protein, 5 aa, Artificial Sequence
  Synthetic Polypeptide
NYIIH

SEQ ID NO: 25 - protein, 5 aa, Artificial Sequence
  Synthetic Polypeptide
NYLIH

SEQ ID NO: 26 - protein, 17 aa, Artificial Sequence
  Synthetic Polypeptide
WIYPGNVYIQYSQKFQG

SEQ ID NO: 27 - protein, 17 aa, Artificial Sequence
  Synthetic Polypeptide
WIYPGDVYIQYNEKFKG

SEQ ID NO: 28 - protein, 17 aa, Artificial Sequence
  Synthetic Polypeptide
WFYPGNVYIQYNEKFKG

SEQ ID NO: 29 - protein, 17 aa, Artificial Sequence
  Synthetic Polypeptide
WINPGNVYIQYNEKFKG

SEQ ID NO: 30 - protein, 7 aa, Artificial Sequence
  Synthetic Polypeptide
EGPWFAY

SEQ ID NO: 31 - protein, 7 aa, Artificial Sequence
  Synthetic Polypeptide
DGPYFAY

SEQ ID NO: 32 - protein, 7 aa, Artificial Sequence
  Synthetic Polypeptide
DGAWFAY

SEQ ID NO: 33 - protein, 7 aa, Artificial Sequence
  Synthetic Polypeptide
DGYWFAY

SEQ ID NO: 34 - protein, 7 aa, Artificial Sequence
  Synthetic Polypeptide
DGSWFAY

SEQ ID NO: 35 - protein, 7 aa, Artificial Sequence
  Synthetic Polypeptide
DGFWFAY

SEQ ID NO: 36 - protein, 7 aa, Artificial Sequence
  Synthetic Polypeptide
DGGWFAY

SEQ ID NO: 37 - protein, 7 aa, Artificial Sequence
  Synthetic Polypeptide
DGTWFAY

SEQ ID NO: 38 - protein, 7 aa, Artificial Sequence
  Synthetic Polypeptide
DGVWFAY

SEQ ID NO: 39 - protein, 16 aa, Artificial Sequence
  Synthetic Polypeptide
RSSKSLLHSDGFTYLY

SEQ ID NO: 40 - protein, 7 aa, Artificial Sequence
  Synthetic Polypeptide
QTSNLAS

SEQ ID NO: 41 - protein, 9 aa, Artificial Sequence
  Synthetic Polypeptide
AQNLELPNT

SEQ ID NO: 42 - protein, 16 aa, Artificial Sequence
  Synthetic Polypeptide
RSSRSLLHSDGFTYLY

SEQ ID NO: 43 - protein, 16 aa, Artificial Sequence
  Synthetic Polypeptide
RSSRSLLHSNGFTYLY

SEQ ID NO: 44 - protein, 16 aa, Artificial Sequence
  Synthetic Polypeptide
RSSRSLLHSDGITYLY

SEQ ID NO: 45 - protein, 16 aa, Artificial Sequence
  Synthetic Polypeptide
RSSRSLLHSDGFTYLS

SEQ ID NO: 46 - protein, 9 aa, Artificial Sequence
  Synthetic Polypeptide
AQNLELPWT

SEQ ID NO: 47 - protein, 9 aa, Artificial Sequence
  Synthetic Polypeptide
QQNLELPNT

SEQ ID NO: 48 - protein, 9 aa, Artificial Sequence
  Synthetic Polypeptide
LQNLELPNT

SEQ ID NO: 49 - protein, 9 aa, Artificial Sequence
  Synthetic Polypeptide
AQYLELPNT

SEQ ID NO: 50 - protein, 9 aa, Artificial Sequence
  Synthetic Polypeptide
AQGLELPNT

SEQ ID NO: 51 - protein, 9 aa, Artificial Sequence
  Synthetic Polypeptide
AQSLELPNT

SEQ ID NO: 52 - protein, 116 aa, Artificial Sequence
  Synthetic Polypeptide
EVKLEESGPALVKPGASVRISCKASGYTFTNYYIHWVKQRPGQGLDYIGWIYPGNVYIQYNEKFKGKATLTADKSSSTAFMQLSSLTSEDSAVYFCARDGPWFAYWGQGTLVTVSS

SEQ ID NO: 53 - protein, 116 aa, Artificial Sequence
  Synthetic Polypeptide
QVQLVQSGAEVKKPGASVKVSCKASGYTFTNYYIHWVRQAPGQRLEWMGWIYPGNVYIQYSQKFQGRVTITRDTSASTAYMELSSLRSEDTAVYYCARDGPWFAYWGQGTLVTVSS

SEQ ID NO: 54 - protein, 116 aa, Artificial Sequence
  Synthetic Polypeptide
QVQLVQSGAEVKKPGASVKVSCKASGYTFTNYYIHWVRQAPGQRLEYIGWIYPGNVYIQYNEKFKGRATLTADKSASTAYMELSSLRSEDTAVYYCARDGPWFAYWGQGTLVTVSS

SEQ ID NO: 55 - protein, 116 aa, Artificial Sequence
  Synthetic Polypeptide
QVQLVQSGAEVKKPGASVKVSCKASGYTFTNYYIHWVRQAPGQRLEWMGWIYPGNVYIQYNEKFKGRVTITRDTSASTAYMELSSLRSEDTAVYYCARDGPWFAYWGQGTLVTVSS

SEQ ID NO: 56 - protein, 116 aa, Artificial Sequence
  Synthetic Polypeptide
QVQLVQSGAEVKKPGASVKVSCKASGYTFTNYYIHWVRQAPGQRLEYIGWIYPGNVYIQYSQKFQGRVTITADKSASTAYMELSSLRSEDTAVYYCARDGPWFAYWGQGTLVTVSS

SEQ ID NO: 57 - protein, 116 aa, Artificial Sequence
  Synthetic Polypeptide
QVQLVESGAEVKKPGASVKVSCKASGYTFTNYYIHWVRQAPGQRLEYIGWIYPGNVYIQYNEKFKGRATLTADKSASTAYMELSSLRSEDTAVYYCARDGPWFAYWGQGTLVTVSS

SEQ ID NO: 58 - protein, 116 aa, Artificial Sequence
  Synthetic Polypeptide
QVQLVQSGAEVKKPGASVKVSCKASGYTFTSYYIHWVRQAPGQRLEYIGWIYPGNVYIQYNEKFKGRATLTADKSASTAYMELSSLRSEDTAVYYCARDGPWFAYWGQGTLVTVSS

SEQ ID NO: 59 - protein, 116 aa, Artificial Sequence
  Synthetic Polypeptide
QVQLVQSGAEVKKPGASVKVSCKASGYTFTNYNIHWVRQAPGQRLEYIGWIYPGNVYIQYNEKFKGRATLTADKSASTAYMELSSLRSEDTAVYYCARDGPWFAYWGQGTLVTVSS

SEQ ID NO: 60 - protein, 116 aa, Artificial Sequence
  Synthetic Polypeptide
QVQLVQSGAEVKKPGASVKVSCKASGYTFTNYYIHWVRQAPGQRLEYIGWIYPGDVYIQYNEKFKGRATLTADKSASTAYMELSSLRSEDTAVYYCARDGPWFAYWGQGTLVTVSS

SEQ ID NO: 61 - protein, 116 aa, Artificial Sequence
  Synthetic Polypeptide
QVQLVQSGAEVKKPGASVKVSCKASGYTFTNYFIHWVRQAPGQRLEYIGWIYPGNVYIQYNEKFKGRATLTADKSASTAYMELSSLRSEDTAVYYCARDGPWFAYWGQGTLVTVSS

SEQ ID NO: 62 - protein, 116 aa, Artificial Sequence
  Synthetic Polypeptide
QVQLVQSGAEVKKPGASVKVSCKASGYTFTNYSIHWVRQAPGQRLEYIGWIYPGNVYIQYNEKFKGRATLTADKSASTAYMELSSLRSEDTAVYYCARDGPWFAYWGQGTLVTVSS

SEQ ID NO: 63 - protein, 116 aa, Artificial Sequence
  Synthetic Polypeptide
QVQLVQSGAEVKKPGASVKVSCKASGYTFTNYWIHWVRQAPGQRLEYIGWIYPGNVYIQYNEKFKGRATLTADKSASTAYMELSSLRSEDTAVYYCARDGPWFAYWGQGTLVTVSS

SEQ ID NO: 64 - protein, 116 aa, Artificial Sequence
  Synthetic Polypeptide
QVQLVQSGAEVKKPGASVKVSCKASGYTFTNYYIHWVRQAPGQRLEYIGWFYPGNVYIQYNEKFKGRATLTADKSASTAYMELSSLRSEDTAVYYCARDGPWFAYWGQGTLVTVSS

SEQ ID NO: 65 - protein, 116 aa, Artificial Sequence
  Synthetic Polypeptide
QVQLVQSGAEVKKPGASVKVSCKASGYTFTNYYIHWVRQAPGQRLEWIGWIYPGNVYIQYNEKFKGRATLTADKSASTAYMELSSLRSEDTAVYYCARDGPWFAYWGQGTLVTVSS

SEQ ID NO: 66 - protein, 116 aa, Artificial Sequence
  Synthetic Polypeptide
QVQLVQSGAEVKKPGASVKVSCKASGYTFTNYYIHWVRQAPGQRLEYIGWINPGNVYIQYNEKFKGRATLTADKSASTAYMELSSLRSEDTAVYYCARDGPWFAYWGQGTLVTVSS

SEQ ID NO: 67 - protein, 116 aa, Artificial Sequence
  Synthetic Polypeptide
QVQLVQSGAEVKKPGASVKVSCKASGYTFTNYYIHWVRQAPGQRLEYIGWIYPGNVYIQYNEKFKGRATLTADKSASTAYMELSSLRSEDTAVYYCAREGPWFAYWGQGTLVTVSS

SEQ ID NO: 68 - protein, 116 aa, Artificial Sequence
  Synthetic Polypeptide
QVQLVQSGAEVKKPGASVKVSCKASGYTFTNYYIHWVRQAPGQRLEYIGWIYPGNVYIQYNEKFKGRATLTADKSASTAYMELSSLRSEDTAVYYCARDGPYFAYWGQGTLVTVSS

SEQ ID NO: 69 - protein, 116 aa, Artificial Sequence
  Synthetic Polypeptide
QVQLVQSGAEVKKPGASVKVSCKASGYTFTNYYIHWVRQAPGQRLEYIGWIYPGNVYIQYNEKFKGRATLTADKSASTAYMELSSLRSEDTAVYYCARDGAWFAYWGQGTLVTVSS

SEQ ID NO: 70 - protein, 116 aa, Artificial Sequence
  Synthetic Polypeptide
QVQLVQSGAEVKKPGASVKVSCKASGYTFTNYYMHWVRQAPGQRLEYIGWIYPGNVYIQYNEKFKGRATLTADKSASTAYMELSSLRSEDTAVYYCARDGPWFAYWGQGTLVTVSS

SEQ ID NO: 71 - protein, 116 aa, Artificial Sequence
  Synthetic Polypeptide
QVQLVQSGAEVKKPGASVKVSCKASGYTFTNYYIHWVRQAPGQRLEYIGWVYPGNVYIQYNEKFKGRATLTADKSASTAYMELSSLRSEDTAVYYCARDGPWFAYWGQGTLVTVSS

SEQ ID NO: 72 - protein, 116 aa, Artificial Sequence
  Synthetic Polypeptide
QVQLVQSGAEVKKPGASVKVSCKASGYTFTNYYIHWVRQAPGQRLEYIGWIYPGNVYIQYNEKFKGRATITADKSASTAYMELSSLRSEDTAVYYCARDGPWFAYWGQGTLVTVSS

SEQ ID NO: 73 - protein, 116 aa, Artificial Sequence
  Synthetic Polypeptide
QVQLVQSGAEVKKPGASVKVSCKASGYTFTNYYIHWVRQAPGQRLEYIGWIYPGNVYIQYNEKFKGRATLTRDKSASTAYMELSSLRSEDTAVYYCARDGPWFAYWGQGTLVTVSS

SEQ ID NO: 74 - protein, 116 aa, Artificial Sequence
  Synthetic Polypeptide
QVQLVQSGAEVKKPGASVKVSCKASGYTFTNYYIHWVRQAPGQRLEYIGWIYPGNVYIQYNEKFKGRVTLTADKSASTAYMELSSLRSEDTAVYYCARDGPWFAYWGQGTLVTVSS

SEQ ID NO: 75 - protein, 116 aa, Artificial Sequence
  Synthetic Polypeptide
QVQLVQSGAEVKKPGASVKVSCKASGYTFTNYHIHWVRQAPGQRLEYIGWIYPGNVYIQYNEKFKGRATLTADKSASTAYMELSSLRSEDTAVYYCARDGPWFAYWGQGTLVTVSS

SEQ ID NO: 76 - protein, 116 aa, Artificial Sequence
  Synthetic Polypeptide
QVQLVQSGAEVKKPGASVKVSCKASGYTFTNYDIHWVRQAPGQRLEYIGWIYPGNVYIQYNEKFKGRATLTADKSASTAYMELSSLRSEDTAVYYCARDGPWFAYWGQGTLVTVSS

SEQ ID NO: 77 - protein, 116 aa, Artificial Sequence
  Synthetic Polypeptide
QVQLVQSGAEVKKPGASVKVSCKASGYTFTNYYIHWVRQAPGQRLEYIGWIYPGNVYIQYNEKFKGRATLTADKSASTAYMELSSLRSEDTAVYYCARDGYWFAYWGQGTLVTVSS

SEQ ID NO: 78 - protein, 116 aa, Artificial Sequence
  Synthetic Polypeptide
QVQLVQSGAEVKKPGASVKVSCKASGYTFTNYYIHWVRQAPGQRLEYIGWIYPGNVYIQYNEKFKGRATLTADKSASTAYMELSSLRSEDTAVYYCARDGSWFAYWGQGTLVTVSS

SEQ ID NO: 79 - protein, 116 aa, Artificial Sequence
  Synthetic Polypeptide
QVQLVQSGAEVKKPGASVKVSCKASGYTFTNYYIHWVRQAPGQRLEYIGWIYPGNVYIQYNEKFKGRATLTADKSASTAYMELSSLRSEDTAVYYCARDGFWFAYWGQGTLVTVSS

SEQ ID NO: 80 - protein, 116 aa, Artificial Sequence
  Synthetic Polypeptide
QVQLVQSGAEVKKPGASVKVSCKASGYTFTNYYIHWVRQAPGQRLEYIGWIYPGNVYIQYNEKFKGRATLTADKSASTAYMELSSLRSEDTAVYYCARDGGWFAYWGQGTLVTVSS

SEQ ID NO: 81 - protein, 116 aa, Artificial Sequence
  Synthetic Polypeptide
QVQLVQSGAEVKKPGASVKVSCKASGYTFTNYYIHWVRQAPGQRLEYIGWIYPGNVYIQYNEKFKGRATLTADKSASTAYMELSSLRSEDTAVYYCARDGTWFAYWGQGTLVTVSS

SEQ ID NO: 82 - protein, 116 aa, Artificial Sequence
  Synthetic Polypeptide
QVQLVQSGAEVKKPGASVKVSCKASGYTFTNYYIHWVRQAPGQRLEYIGWIYPGNVYIQYNEKFKGRATLTADKSASTAYMELSSLRSEDTAVYYCARDGVWFAYWGQGTLVTVSS

SEQ ID NO: 83 - protein, 116 aa, Artificial Sequence
  Synthetic Polypeptide
QVQLVQSGAEVKKPGASVKVSCKASGYTFTNYIIHWVRQAPGQRLEYIGWIYPGNVYIQYNEKFKGRATLTADKSASTAYMELSSLRSEDTAVYYCARDGPWFAYWGQGTLVTVSS

SEQ ID NO: 84 - protein, 116 aa, Artificial Sequence
  Synthetic Polypeptide
QVQLVQSGAEVKKPGASVKVSCKASGYTFTNYLIHWVRQAPGQRLEYIGWIYPGNVYIQYNEKFKGRATLTADKSASTAYMELSSLRSEDTAVYYCARDGPWFAYWGQGTLVTVSS

SEQ ID NO: 85 - protein, 112 aa, Artificial Sequence
  Synthetic Polypeptide
DIVLTQTPFSNPVTLGTSASISCRSSKSLLHSDGFTYLYWFLQKPGQSPHLLIYQTSNLASGVPDRFSSSGSGTDFTLRISRVEAEDVGVYYCAQNLELPNTFGGGTKLEIK

SEQ ID NO: 86 - protein, 112 aa, Artificial Sequence
  Synthetic Polypeptide
DIVMTQTPLSLSVTPGQPASISCRSSRSLLHSDGFTYLYWYLQKPGQSPQLLIYQTSNLASGVPDRFSGSGSGTDFTLKISRVEAEDVGVYYCAQNLELPNTFGQGTKLEIK

SEQ ID NO: 87 - protein, 112 aa, Artificial Sequence
  Synthetic Polypeptide
DIVLTQTPLSLSVTPGQPASISCRSSKSLLHSDGFTYLYWFLQKPGQSPQLLIYQTSNLASGVPDRFSSSGSGTDFTLKISRVEAEDVGVYYCAQNLELPNTFGQGTKLEIK

SEQ ID NO: 88 - protein, 112 aa, Artificial Sequence
  Synthetic Polypeptide
DIVMTQTPLSLSVTPGQPASISCRSSKSLLHSDGFTYLYWFLQKPGQSPQLLIYQTSNLASGVPDRFSGSGSGTDFTLKISRVEAEDVGVYYCAQNLELPNTFGQGTKLEIK

SEQ ID NO: 89 - protein, 112 aa, Artificial Sequence
  Synthetic Polypeptide
DIVLTQTPLSLSVTPGQPASISCRSSRSLLHSDGFTYLYWFLQKPGQSPQLLIYQTSNLASGVPDRFSSSGSGTDFTLKISRVEAEDVGVYYCAQNLELPNTFGQGTKLEIK

SEQ ID NO: 90 - protein, 112 aa, Artificial Sequence
  Synthetic Polypeptide
DIVLTQTPLSLSVTPGQPASISCRSSRSLLHSNGFTYLYWFLQKPGQSPQLLIYQTSNLASGVPDRFSSSGSGTDFTLKISRVEAEDVGVYYCAQNLELPNTFGQGTKLEIK

SEQ ID NO: 91 - protein, 112 aa, Artificial Sequence
  Synthetic Polypeptide
DIVLTQTPLSLSVTPGQPASISCRSSRSLLHSDGITYLYWFLQKPGQSPQLLIYQTSNLASGVPDRFSSSGSGTDFTLKISRVEAEDVGVYYCAQNLELPNTFGQGTKLEIK

SEQ ID NO: 92 - protein, 112 aa, Artificial Sequence
  Synthetic Polypeptide
DIVLTQTPLSLSVTPGQPASISCRSSRSLLHSDGFTYLYWFLQKPGQSPQLLIYQTSNLASGVPDRFSSSGSGTDFTLKISRVEAEDVGVYYCAQNLELPWTFGQGTKLEIK

SEQ ID NO: 93 - protein, 112 aa, Artificial Sequence
  Synthetic Polypeptide
DIVLTQTPLSLSVTPGQPASISCRSSRSLLHSDGFTYLSWFLQKPGQSPQLLIYQTSNLASGVPDRFSSSGSGTDFTLKISRVEAEDVGVYYCAQNLELPNTFGQGTKLEIK

SEQ ID NO: 94 - protein, 112 aa, Artificial Sequence
  Synthetic Polypeptide
DIVLTQTPLSLSVTPGQPASISCRSSRSLLHSDGFTYLYWYLQKPGQSPQLLIYQTSNLASGVPDRFSSSGSGTDFTLKISRVEAEDVGVYYCAQNLELPNTFGQGTKLEIK

SEQ ID NO: 95 - protein, 112 aa, Artificial Sequence
  Synthetic Polypeptide
DIVLTQTPLSLSVTPGQPASISCRSSRSLLHSDGFTYLYWFLQKPGQSPQLLIYQTSNLASGVPDRFSSSGSGTDFTLKISRVEAEDVGVYYCQQNLELPNTFGQGTKLEIK

SEQ ID NO: 96 - protein, 112 aa, Artificial Sequence
  Synthetic Polypeptide
DIVLTQTPLSLSVTPGQPASISCRSSRSLLHSDGFTYLYWFLQKPGQSPQLLIYQTSNLASGVPDRFSSSGSGTDFTLKISRVEAEDVGVYYCLQNLELPNTFGQGTKLEIK

SEQ ID NO: 97 - protein, 112 aa, Artificial Sequence
  Synthetic Polypeptide
DIVLTQTPLSLSVTPGQPASISCRSSRSLLHSDGFTYLYWFLQKPGQSPQLLIYQTSNLASGVPDRFSSSGSGTDFTLKISRVEAEDVGVYYCAQYLELPNTFGQGTKLEIK

SEQ ID NO: 98 - protein, 112 aa, Artificial Sequence
  Synthetic Polypeptide
DIVLTQTPLSLSVTPGQPASISCRSSRSLLHSDGFTYLYWFLQKPGQSPQLLIYQTSNLASGVPDRFSSSGSGTDFTLKISRVEAEDVGVYYCAQGLELPNTFGQGTKLEIK

SEQ ID NO: 99 - protein, 112 aa, Artificial Sequence
  Synthetic Polypeptide
DIVLTQTPLSLSVTPGQPASISCRSSRSLLHSDGFTYLYWFLQKPGQSPQLLIYQTSNLASGVPDRFSSSGSGTDFTLKISRVEAEDVGVYYCAQSLELPNTFGQGTKLEIK

SEQ ID NO: 100 - protein, 452 aa, Artificial Sequence
  Synthetic Polypeptide
EVKLEESGPALVKPGASVRISCKASGYTFTNYYIHWVKQRPGQGLDYIGWIYPGNVYIQYNEKFKGKATLTADKSSSTAFMQLSSLTSEDSAVYFCARDGPWFAYWGQGTLVTVSSAKTTPPSVYPLAPGCGDTTGSSVTLGCLVKGYFPESVTVTWNSGSLSSSVHTFPALLQSGLYTMSSSVTVPSSTWPSQTVTCSVAHPASSTTVDKKLEPSGPISTINPCPPCKECHKCPAPNLEGGPSVFIFPPNIKDVLMISLTPKVTCVVVDVSEDDPDVRISWFVNNVEVHTAQTQTHREDYNSTIRVVSALPIQHQDWMSGKEFKCKVNNKDLPSPIERTISKIKGLVRAPQVYILPPPAEQLSRKDVSLTCLVVGFNPGDISVEWTSNGHTEENYKDTAPVLDSDGSYFIYSKLDIKTSKWEKTDSFSCNVRHEGLKNYYLKKTISRSPGK

SEQ ID NO: 101 - protein, 445 aa, Artificial Sequence
  Synthetic Polypeptide
EVKLEESGPALVKPGASVRISCKASGYTFTNYYIHWVKQRPGQGLDYIGWIYPGNVYIQYNEKFKGKATLTADKSSSTAFMQLSSLTSEDSAVYFCARDGPWFAYWGQGTLVTVSSASTKGPSVFPLAPSSKSTSGGTAALGCLVKDYFPEPVTVSWNSGALTSGVHTFPAVLQSSGLYSLSSVVTVPSSSLGTQTYICNVNHKPSNTKVDKKVEPKSCDKTHTCPPCPAPELLGGPSVFLFPPKPKDTLMISRTPEVTCVVVDVSHEDPEVKFNWYVDGVEVHNAKTKPREEQYNSTYRVVSVLTVLHQDWLNGKEYKCKVSNKALPAPIEKTISKAKGQPREPQVYTLPPSRDELTKNQVSLTCLVKGFYPSDIAVEWESNGQPENNYKTTPPVLDSDGSFFLYSKLTVDKSRWQQGNVFSCSVMHEALHNHYTQKSLSLSPG

SEQ ID NO: 102 - protein, 445 aa, Artificial Sequence
  Synthetic Polypeptide
QVQLVQSGAEVKKPGASVKVSCKASGYTFTNYYIHWVRQAPGQRLEWMGWIYPGNVYIQYSQKFQGRVTITRDTSASTAYMELSSLRSEDTAVYYCARDGPWFAYWGQGTLVTVSSASTKGPSVFPLAPSSKSTSGGTAALGCLVKDYFPEPVTVSWNSGALTSGVHTFPAVLQSSGLYSLSSVVTVPSSSLGTQTYICNVNHKPSNTKVDKKVEPKSCDKTHTCPPCPAPELLGGPSVFLFPPKPKDTLMISRTPEVTCVVVDVSHEDPEVKFNWYVDGVEVHNAKTKPREEQYNSTYRVVSVLTVLHQDWLNGKEYKCKVSNKALPAPIEKTISKAKGQPREPQVYTLPPSRDELTKNQVSLTCLVKGFYPSDIAVEWESNGQPENNYKTTPPVLDSDGSFFLYSKLTVDKSRWQQGNVFSCSVMHEALHNHYTQKSLSLSPG

SEQ ID NO: 103 - protein, 445 aa, Artificial Sequence
  Synthetic Polypeptide
QVQLVQSGAEVKKPGASVKVSCKASGYTFTNYYIHWVRQAPGQRLEYIGWIYPGNVYIQYNEKFKGRATLTADKSASTAYMELSSLRSEDTAVYYCARDGPWFAYWGQGTLVTVSSASTKGPSVFPLAPSSKSTSGGTAALGCLVKDYFPEPVTVSWNSGALTSGVHTFPAVLQSSGLYSLSSVVTVPSSSLGTQTYICNVNHKPSNTKVDKKVEPKSCDKTHTCPPCPAPELLGGPSVFLFPPKPKDTLMISRTPEVTCVVVDVSHEDPEVKFNWYVDGVEVHNAKTKPREEQYNSTYRVVSVLTVLHQDWLNGKEYKCKVSNKALPAPIEKTISKAKGQPREPQVYTLPPSRDELTKNQVSLTCLVKGFYPSDIAVEWESNGQPENNYKTTPPVLDSDGSFFLYSKLTVDKSRWQQGNVFSCSVMHEALHNHYTQKSLSLSPG

SEQ ID NO: 104 - protein, 450 aa, Artificial Sequence
  Synthetic Polypeptide
QVQLVQSGAEVKKPGASVKVSCKASGYTFTNYYIHWVRQAPGQRLEYIGWIYPGNVYIQYNEKFKGRATLTADKSASTAYMELSSLRSEDTAVYYCARDGPWFAYWGQGTLVTVSSASTKGPSVFPLAPSSKSTSGGTAALGCLVKDYFPEPVTVSWNSGALTSGVHTFPAVLQSSGLYSLSSVVTVPSSSLGTQTYICNVNHKPSNTKVDKKVEPKSCDKTHTCPPCPAPELLGGPSVFLFPPKPKDTLMISRTPEVTCVVVDVSHEDPEVKFNWYVDGVEVHNAKTKPREEQYNSTYRVVSVLTVLHQDWLNGKEYKCKVSNKALPAPIEKTISKAKGQPREPQVYTLPPSRDELTKNQVSLTCLVKGFYPSDIAVEWESNGQPENNYKTTPPVLDSDGSFFLYSKLTVDKSRWQQGNVFSCSVMHEALHNHYTQKSLCLSPGSLSPG

SEQ ID NO: 105 - protein, 445 aa, Artificial Sequence
  Synthetic Polypeptide
QVQLVQSGAEVKKPGASVKVSCKASGYTFTNYYIHWVRQAPGQRLEWMGWIYPGNVYIQYNEKFKGRVTITRDTSASTAYMELSSLRSEDTAVYYCARDGPWFAYWGQGTLVTVSSASTKGPSVFPLAPSSKSTSGGTAALGCLVKDYFPEPVTVSWNSGALTSGVHTFPAVLQSSGLYSLSSVVTVPSSSLGTQTYICNVNHKPSNTKVDKKVEPKSCDKTHTCPPCPAPELLGGPSVFLFPPKPKDTLMISRTPEVTCVVVDVSHEDPEVKFNWYVDGVEVHNAKTKPREEQYNSTYRVVSVLTVLHQDWLNGKEYKCKVSNKALPAPIEKTISKAKGQPREPQVYTLPPSRDELTKNQVSLTCLVKGFYPSDIAVEWESNGQPENNYKTTPPVLDSDGSFFLYSKLTVDKSRWQQGNVFSCSVMHEALHNHYTQKSLSLSPG

SEQ ID NO: 106 - protein, 445 aa, Artificial Sequence
  Synthetic Polypeptide
QVQLVQSGAEVKKPGASVKVSCKASGYTFTNYYIHWVRQAPGQRLEYIGWIYPGNVYIQYSQKFQGRVTITADKSASTAYMELSSLRSEDTAVYYCARDGPWFAYWGQGTLVTVSSASTKGPSVFPLAPSSKSTSGGTAALGCLVKDYFPEPVTVSWNSGALTSGVHTFPAVLQSSGLYSLSSVVTVPSSSLGTQTYICNVNHKPSNTKVDKKVEPKSCDKTHTCPPCPAPELLGGPSVFLFPPKPKDTLMISRTPEVTCVVVDVSHEDPEVKFNWYVDGVEVHNAKTKPREEQYNSTYRVVSVLTVLHQDWLNGKEYKCKVSNKALPAPIEKTISKAKGQPREPQVYTLPPSRDELTKNQVSLTCLVKGFYPSDIAVEWESNGQPENNYKTTPPVLDSDGSFFLYSKLTVDKSRWQQGNVFSCSVMHEALHNHYTQKSLSLSPG

SEQ ID NO: 107 - protein, 445 aa, Artificial Sequence
  Synthetic Polypeptide
QVQLVESGAEVKKPGASVKVSCKASGYTFTNYYIHWVRQAPGQRLEYIGWIYPGNVYIQYNEKFKGRATLTADKSASTAYMELSSLRSEDTAVYYCARDGPWFAYWGQGTLVTVSSASTKGPSVFPLAPSSKSTSGGTAALGCLVKDYFPEPVTVSWNSGALTSGVHTFPAVLQSSGLYSLSSVVTVPSSSLGTQTYICNVNHKPSNTKVDKKVEPKSCDKTHTCPPCPAPELLGGPSVFLFPPKPKDTLMISRTPEVTCVVVDVSHEDPEVKFNWYVDGVEVHNAKTKPREEQYNSTYRVVSVLTVLHQDWLNGKEYKCKVSNKALPAPIEKTISKAKGQPREPQVYTLPPSRDELTKNQVSLTCLVKGFYPSDIAVEWESNGQPENNYKTTPPVLDSDGSFFLYSKLTVDKSRWQQGNVFSCSVMHEALHNHYTQKSLSLSPG

SEQ ID NO: 108 - protein, 445 aa, Artificial Sequence
  Synthetic Polypeptide
QVQLVQSGAEVKKPGASVKVSCKASGYTFTSYYIHWVRQAPGQRLEYIGWIYPGNVYIQYNEKFKGRATLTADKSASTAYMELSSLRSEDTAVYYCARDGPWFAYWGQGTLVTVSSASTKGPSVFPLAPSSKSTSGGTAALGCLVKDYFPEPVTVSWNSGALTSGVHTFPAVLQSSGLYSLSSVVTVPSSSLGTQTYICNVNHKPSNTKVDKKVEPKSCDKTHTCPPCPAPELLGGPSVFLFPPKPKDTLMISRTPEVTCVVVDVSHEDPEVKFNWYVDGVEVHNAKTKPREEQYNSTYRVVSVLTVLHQDWLNGKEYKCKVSNKALPAPIEKTISKAKGQPREPQVYTLPPSRDELTKNQVSLTCLVKGFYPSDIAVEWESNGQPENNYKTTPPVLDSDGSFFLYSKLTVDKSRWQQGNVFSCSVMHEALHNHYTQKSLSLSPG

SEQ ID NO: 109 - protein, 445 aa, Artificial Sequence
  Synthetic Polypeptide
QVQLVQSGAEVKKPGASVKVSCKASGYTFTNYNIHWVRQAPGQRLEYIGWIYPGNVYIQYNEKFKGRATLTADKSASTAYMELSSLRSEDTAVYYCARDGPWFAYWGQGTLVTVSSASTKGPSVFPLAPSSKSTSGGTAALGCLVKDYFPEPVTVSWNSGALTSGVHTFPAVLQSSGLYSLSSVVTVPSSSLGTQTYICNVNHKPSNTKVDKKVEPKSCDKTHTCPPCPAPELLGGPSVFLFPPKPKDTLMISRTPEVTCVVVDVSHEDPEVKFNWYVDGVEVHNAKTKPREEQYNSTYRVVSVLTVLHQDWLNGKEYKCKVSNKALPAPIEKTISKAKGQPREPQVYTLPPSRDELTKNQVSLTCLVKGFYPSDIAVEWESNGQPENNYKTTPPVLDSDGSFFLYSKLTVDKSRWQQGNVFSCSVMHEALHNHYTQKSLSLSPG

SEQ ID NO: 110 - protein, 445 aa, Artificial Sequence
  Synthetic Polypeptide
QVQLVQSGAEVKKPGASVKVSCKASGYTFTNYYIHWVRQAPGQRLEYIGWIYPGDVYIQYNEKFKGRATLTADKSASTAYMELSSLRSEDTAVYYCARDGPWFAYWGQGTLVTVSSASTKGPSVFPLAPSSKSTSGGTAALGCLVKDYFPEPVTVSWNSGALTSGVHTFPAVLQSSGLYSLSSVVTVPSSSLGTQTYICNVNHKPSNTKVDKKVEPKSCDKTHTCPPCPAPELLGGPSVFLFPPKPKDTLMISRTPEVTCVVVDVSHEDPEVKFNWYVDGVEVHNAKTKPREEQYNSTYRVVSVLTVLHQDWLNGKEYKCKVSNKALPAPIEKTISKAKGQPREPQVYTLPPSRDELTKNQVSLTCLVKGFYPSDIAVEWESNGQPENNYKTTPPVLDSDGSFFLYSKLTVDKSRWQQGNVFSCSVMHEALHNHYTQKSLSLSPG

SEQ ID NO: 111 - protein, 445 aa, Artificial Sequence
  Synthetic Polypeptide
QVQLVQSGAEVKKPGASVKVSCKASGYTFTNYFIHWVRQAPGQRLEYIGWIYPGNVYIQYNEKFKGRATLTADKSASTAYMELSSLRSEDTAVYYCARDGPWFAYWGQGTLVTVSSASTKGPSVFPLAPSSKSTSGGTAALGCLVKDYFPEPVTVSWNSGALTSGVHTFPAVLQSSGLYSLSSVVTVPSSSLGTQTYICNVNHKPSNTKVDKKVEPKSCDKTHTCPPCPAPELLGGPSVFLFPPKPKDTLMISRTPEVTCVVVDVSHEDPEVKFNWYVDGVEVHNAKTKPREEQYNSTYRVVSVLTVLHQDWLNGKEYKCKVSNKALPAPIEKTISKAKGQPREPQVYTLPPSRDELTKNQVSLTCLVKGFYPSDIAVEWESNGQPENNYKTTPPVLDSDGSFFLYSKLTVDKSRWQQGNVFSCSVMHEALHNHYTQKSLSLSPG

SEQ ID NO: 112 - protein, 445 aa, Artificial Sequence
  Synthetic Polypeptide
QVQLVQSGAEVKKPGASVKVSCKASGYTFTNYSIHWVRQAPGQRLEYIGWIYPGNVYIQYNEKFKGRATLTADKSASTAYMELSSLRSEDTAVYYCARDGPWFAYWGQGTLVTVSSASTKGPSVFPLAPSSKSTSGGTAALGCLVKDYFPEPVTVSWNSGALTSGVHTFPAVLQSSGLYSLSSVVTVPSSSLGTQTYICNVNHKPSNTKVDKKVEPKSCDKTHTCPPCPAPELLGGPSVFLFPPKPKDTLMISRTPEVTCVVVDVSHEDPEVKFNWYVDGVEVHNAKTKPREEQYNSTYRVVSVLTVLHQDWLNGKEYKCKVSNKALPAPIEKTISKAKGQPREPQVYTLPPSRDELTKNQVSLTCLVKGFYPSDIAVEWESNGQPENNYKTTPPVLDSDGSFFLYSKLTVDKSRWQQGNVFSCSVMHEALHNHYTQKSLSLSPG

SEQ ID NO: 113 - protein, 445 aa, Artificial Sequence
  Synthetic Polypeptide
QVQLVQSGAEVKKPGASVKVSCKASGYTFTNYWIHWVRQAPGQRLEYIGWIYPGNVYIQYNEKFKGRATLTADKSASTAYMELSSLRSEDTAVYYCARDGPWFAYWGQGTLVTVSSASTKGPSVFPLAPSSKSTSGGTAALGCLVKDYFPEPVTVSWNSGALTSGVHTFPAVLQSSGLYSLSSVVTVPSSSLGTQTYICNVNHKPSNTKVDKKVEPKSCDKTHTCPPCPAPELLGGPSVFLFPPKPKDTLMISRTPEVTCVVVDVSHEDPEVKFNWYVDGVEVHNAKTKPREEQYNSTYRVVSVLTVLHQDWLNGKEYKCKVSNKALPAPIEKTISKAKGQPREPQVYTLPPSRDELTKNQVSLTCLVKGFYPSDIAVEWESNGQPENNYKTTPPVLDSDGSFFLYSKLTVDKSRWQQGNVFSCSVMHEALHNHYTQKSLSLSPG

SEQ ID NO: 114 - protein, 445 aa, Artificial Sequence
  Synthetic Polypeptide
QVQLVQSGAEVKKPGASVKVSCKASGYTFTNYYIHWVRQAPGQRLEYIGWFYPGNVYIQYNEKFKGRATLTADKSASTAYMELSSLRSEDTAVYYCARDGPWFAYWGQGTLVTVSSASTKGPSVFPLAPSSKSTSGGTAALGCLVKDYFPEPVTVSWNSGALTSGVHTFPAVLQSSGLYSLSSVVTVPSSSLGTQTYICNVNHKPSNTKVDKKVEPKSCDKTHTCPPCPAPELLGGPSVFLFPPKPKDTLMISRTPEVTCVVVDVSHEDPEVKFNWYVDGVEVHNAKTKPREEQYNSTYRVVSVLTVLHQDWLNGKEYKCKVSNKALPAPIEKTISKAKGQPREPQVYTLPPSRDELTKNQVSLTCLVKGFYPSDIAVEWESNGQPENNYKTTPPVLDSDGSFFLYSKLTVDKSRWQQGNVFSCSVMHEALHNHYTQKSLSLSPG

SEQ ID NO: 115 - protein, 445 aa, Artificial Sequence
  Synthetic Polypeptide
QVQLVQSGAEVKKPGASVKVSCKASGYTFTNYYIHWVRQAPGQRLEWIGWIYPGNVYIQYNEKFKGRATLTADKSASTAYMELSSLRSEDTAVYYCARDGPWFAYWGQGTLVTVSSASTKGPSVFPLAPSSKSTSGGTAALGCLVKDYFPEPVTVSWNSGALTSGVHTFPAVLQSSGLYSLSSVVTVPSSSLGTQTYICNVNHKPSNTKVDKKVEPKSCDKTHTCPPCPAPELLGGPSVFLFPPKPKDTLMISRTPEVTCVVVDVSHEDPEVKFNWYVDGVEVHNAKTKPREEQYNSTYRVVSVLTVLHQDWLNGKEYKCKVSNKALPAPIEKTISKAKGQPREPQVYTLPPSRDELTKNQVSLTCLVKGFYPSDIAVEWESNGQPENNYKTTPPVLDSDGSFFLYSKLTVDKSRWQQGNVFSCSVMHEALHNHYTQKSLSLSPG

SEQ ID NO: 116 - protein, 445 aa, Artificial Sequence
  Synthetic Polypeptide
QVQLVQSGAEVKKPGASVKVSCKASGYTFTNYYIHWVRQAPGQRLEYIGWINPGNVYIQYNEKFKGRATLTADKSASTAYMELSSLRSEDTAVYYCARDGPWFAYWGQGTLVTVSSASTKGPSVFPLAPSSKSTSGGTAALGCLVKDYFPEPVTVSWNSGALTSGVHTFPAVLQSSGLYSLSSVVTVPSSSLGTQTYICNVNHKPSNTKVDKKVEPKSCDKTHTCPPCPAPELLGGPSVFLFPPKPKDTLMISRTPEVTCVVVDVSHEDPEVKFNWYVDGVEVHNAKTKPREEQYNSTYRVVSVLTVLHQDWLNGKEYKCKVSNKALPAPIEKTISKAKGQPREPQVYTLPPSRDELTKNQVSLTCLVKGFYPSDIAVEWESNGQPENNYKTTPPVLDSDGSFFLYSKLTVDKSRWQQGNVFSCSVMHEALHNHYTQKSLSLSPG

SEQ ID NO: 117 - protein, 445 aa, Artificial Sequence
  Synthetic Polypeptide
QVQLVQSGAEVKKPGASVKVSCKASGYTFTNYYIHWVRQAPGQRLEYIGWIYPGNVYIQYNEKFKGRATLTADKSASTAYMELSSLRSEDTAVYYCAREGPWFAYWGQGTLVTVSSASTKGPSVFPLAPSSKSTSGGTAALGCLVKDYFPEPVTVSWNSGALTSGVHTFPAVLQSSGLYSLSSVVTVPSSSLGTQTYICNVNHKPSNTKVDKKVEPKSCDKTHTCPPCPAPELLGGPSVFLFPPKPKDTLMISRTPEVTCVVVDVSHEDPEVKFNWYVDGVEVHNAKTKPREEQYNSTYRVVSVLTVLHQDWLNGKEYKCKVSNKALPAPIEKTISKAKGQPREPQVYTLPPSRDELTKNQVSLTCLVKGFYPSDIAVEWESNGQPENNYKTTPPVLDSDGSFFLYSKLTVDKSRWQQGNVFSCSVMHEALHNHYTQKSLSLSPG

SEQ ID NO: 118 - protein, 445 aa, Artificial Sequence
  Synthetic Polypeptide
QVQLVQSGAEVKKPGASVKVSCKASGYTFTNYYIHWVRQAPGQRLEYIGWIYPGNVYIQYNEKFKGRATLTADKSASTAYMELSSLRSEDTAVYYCARDGPYFAYWGQGTLVTVSSASTKGPSVFPLAPSSKSTSGGTAALGCLVKDYFPEPVTVSWNSGALTSGVHTFPAVLQSSGLYSLSSVVTVPSSSLGTQTYICNVNHKPSNTKVDKKVEPKSCDKTHTCPPCPAPELLGGPSVFLFPPKPKDTLMISRTPEVTCVVVDVSHEDPEVKFNWYVDGVEVHNAKTKPREEQYNSTYRVVSVLTVLHQDWLNGKEYKCKVSNKALPAPIEKTISKAKGQPREPQVYTLPPSRDELTKNQVSLTCLVKGFYPSDIAVEWESNGQPENNYKTTPPVLDSDGSFFLYSKLTVDKSRWQQGNVFSCSVMHEALHNHYTQKSLSLSPG

SEQ ID NO: 119 - protein, 445 aa, Artificial Sequence
  Synthetic Polypeptide
QVQLVQSGAEVKKPGASVKVSCKASGYTFTNYYIHWVRQAPGQRLEYIGWIYPGNVYIQYNEKFKGRATLTADKSASTAYMELSSLRSEDTAVYYCARDGAWFAYWGQGTLVTVSSASTKGPSVFPLAPSSKSTSGGTAALGCLVKDYFPEPVTVSWNSGALTSGVHTFPAVLQSSGLYSLSSVVTVPSSSLGTQTYICNVNHKPSNTKVDKKVEPKSCDKTHTCPPCPAPELLGGPSVFLFPPKPKDTLMISRTPEVTCVVVDVSHEDPEVKFNWYVDGVEVHNAKTKPREEQYNSTYRVVSVLTVLHQDWLNGKEYKCKVSNKALPAPIEKTISKAKGQPREPQVYTLPPSRDELTKNQVSLTCLVKGFYPSDIAVEWESNGQPENNYKTTPPVLDSDGSFFLYSKLTVDKSRWQQGNVFSCSVMHEALHNHYTQKSLSLSPG

SEQ ID NO: 120 - protein, 445 aa, Artificial Sequence
  Synthetic Polypeptide
QVQLVQSGAEVKKPGASVKVSCKASGYTFTNYYMHWVRQAPGQRLEYIGWIYPGNVYIQYNEKFKGRATLTADKSASTAYMELSSLRSEDTAVYYCARDGPWFAYWGQGTLVTVSSASTKGPSVFPLAPSSKSTSGGTAALGCLVKDYFPEPVTVSWNSGALTSGVHTFPAVLQSSGLYSLSSVVTVPSSSLGTQTYICNVNHKPSNTKVDKKVEPKSCDKTHTCPPCPAPELLGGPSVFLFPPKPKDTLMISRTPEVTCVVVDVSHEDPEVKFNWYVDGVEVHNAKTKPREEQYNSTYRVVSVLTVLHQDWLNGKEYKCKVSNKALPAPIEKTISKAKGQPREPQVYTLPPSRDELTKNQVSLTCLVKGFYPSDIAVEWESNGQPENNYKTTPPVLDSDGSFFLYSKLTVDKSRWQQGNVFSCSVMHEALHNHYTQKSLSLSPG

SEQ ID NO: 121 - protein, 445 aa, Artificial Sequence
  Synthetic Polypeptide
QVQLVQSGAEVKKPGASVKVSCKASGYTFTNYYIHWVRQAPGQRLEYIGWVYPGNVYIQYNEKFKGRATLTADKSASTAYMELSSLRSEDTAVYYCARDGPWFAYWGQGTLVTVSSASTKGPSVFPLAPSSKSTSGGTAALGCLVKDYFPEPVTVSWNSGALTSGVHTFPAVLQSSGLYSLSSVVTVPSSSLGTQTYICNVNHKPSNTKVDKKVEPKSCDKTHTCPPCPAPELLGGPSVFLFPPKPKDTLMISRTPEVTCVVVDVSHEDPEVKFNWYVDGVEVHNAKTKPREEQYNSTYRVVSVLTVLHQDWLNGKEYKCKVSNKALPAPIEKTISKAKGQPREPQVYTLPPSRDELTKNQVSLTCLVKGFYPSDIAVEWESNGQPENNYKTTPPVLDSDGSFFLYSKLTVDKSRWQQGNVFSCSVMHEALHNHYTQKSLSLSPG

SEQ ID NO: 122 - protein, 445 aa, Artificial Sequence
  Synthetic Polypeptide
QVQLVQSGAEVKKPGASVKVSCKASGYTFTNYYIHWVRQAPGQRLEYIGWIYPGNVYIQYNEKFKGRATITADKSASTAYMELSSLRSEDTAVYYCARDGPWFAYWGQGTLVTVSSASTKGPSVFPLAPSSKSTSGGTAALGCLVKDYFPEPVTVSWNSGALTSGVHTFPAVLQSSGLYSLSSVVTVPSSSLGTQTYICNVNHKPSNTKVDKKVEPKSCDKTHTCPPCPAPELLGGPSVFLFPPKPKDTLMISRTPEVTCVVVDVSHEDPEVKFNWYVDGVEVHNAKTKPREEQYNSTYRVVSVLTVLHQDWLNGKEYKCKVSNKALPAPIEKTISKAKGQPREPQVYTLPPSRDELTKNQVSLTCLVKGFYPSDIAVEWESNGQPENNYKTTPPVLDSDGSFFLYSKLTVDKSRWQQGNVFSCSVMHEALHNHYTQKSLSLSPG

SEQ ID NO: 123 - protein, 445 aa, Artificial Sequence
  Synthetic Polypeptide
QVQLVQSGAEVKKPGASVKVSCKASGYTFTNYYIHWVRQAPGQRLEYIGWIYPGNVYIQYNEKFKGRATLTRDKSASTAYMELSSLRSEDTAVYYCARDGPWFAYWGQGTLVTVSSASTKGPSVFPLAPSSKSTSGGTAALGCLVKDYFPEPVTVSWNSGALTSGVHTFPAVLQSSGLYSLSSVVTVPSSSLGTQTYICNVNHKPSNTKVDKKVEPKSCDKTHTCPPCPAPELLGGPSVFLFPPKPKDTLMISRTPEVTCVVVDVSHEDPEVKFNWYVDGVEVHNAKTKPREEQYNSTYRVVSVLTVLHQDWLNGKEYKCKVSNKALPAPIEKTISKAKGQPREPQVYTLPPSRDELTKNQVSLTCLVKGFYPSDIAVEWESNGQPENNYKTTPPVLDSDGSFFLYSKLTVDKSRWQQGNVFSCSVMHEALHNHYTQKSLSLSPG

SEQ ID NO: 124 - protein, 445 aa, Artificial Sequence
  Synthetic Polypeptide
QVQLVQSGAEVKKPGASVKVSCKASGYTFTNYYIHWVRQAPGQRLEYIGWIYPGNVYIQYNEKFKGRVTLTADKSASTAYMELSSLRSEDTAVYYCARDGPWFAYWGQGTLVTVSSASTKGPSVFPLAPSSKSTSGGTAALGCLVKDYFPEPVTVSWNSGALTSGVHTFPAVLQSSGLYSLSSVVTVPSSSLGTQTYICNVNHKPSNTKVDKKVEPKSCDKTHTCPPCPAPELLGGPSVFLFPPKPKDTLMISRTPEVTCVVVDVSHEDPEVKFNWYVDGVEVHNAKTKPREEQYNSTYRVVSVLTVLHQDWLNGKEYKCKVSNKALPAPIEKTISKAKGQPREPQVYTLPPSRDELTKNQVSLTCLVKGFYPSDIAVEWESNGQPENNYKTTPPVLDSDGSFFLYSKLTVDKSRWQQGNVFSCSVMHEALHNHYTQKSLSLSPG

SEQ ID NO: 125 - protein, 445 aa, Artificial Sequence
  Synthetic Polypeptide
QVQLVQSGAEVKKPGASVKVSCKASGYTFTNYHIHWVRQAPGQRLEYIGWIYPGNVYIQYNEKFKGRATLTADKSASTAYMELSSLRSEDTAVYYCARDGPWFAYWGQGTLVTVSSASTKGPSVFPLAPSSKSTSGGTAALGCLVKDYFPEPVTVSWNSGALTSGVHTFPAVLQSSGLYSLSSVVTVPSSSLGTQTYICNVNHKPSNTKVDKKVEPKSCDKTHTCPPCPAPELLGGPSVFLFPPKPKDTLMISRTPEVTCVVVDVSHEDPEVKFNWYVDGVEVHNAKTKPREEQYNSTYRVVSVLTVLHQDWLNGKEYKCKVSNKALPAPIEKTISKAKGQPREPQVYTLPPSRDELTKNQVSLTCLVKGFYPSDIAVEWESNGQPENNYKTTPPVLDSDGSFFLYSKLTVDKSRWQQGNVFSCSVMHEALHNHYTQKSLSLSPG

SEQ ID NO: 126 - protein, 445 aa, Artificial Sequence
  Synthetic Polypeptide
QVQLVQSGAEVKKPGASVKVSCKASGYTFTNYDIHWVRQAPGQRLEYIGWIYPGNVYIQYNEKFKGRATLTADKSASTAYMELSSLRSEDTAVYYCARDGPWFAYWGQGTLVTVSSASTKGPSVFPLAPSSKSTSGGTAALGCLVKDYFPEPVTVSWNSGALTSGVHTFPAVLQSSGLYSLSSVVTVPSSSLGTQTYICNVNHKPSNTKVDKKVEPKSCDKTHTCPPCPAPELLGGPSVFLFPPKPKDTLMISRTPEVTCVVVDVSHEDPEVKFNWYVDGVEVHNAKTKPREEQYNSTYRVVSVLTVLHQDWLNGKEYKCKVSNKALPAPIEKTISKAKGQPREPQVYTLPPSRDELTKNQVSLTCLVKGFYPSDIAVEWESNGQPENNYKTTPPVLDSDGSFFLYSKLTVDKSRWQQGNVFSCSVMHEALHNHYTQKSLSLSPG

SEQ ID NO: 127 - protein, 445 aa, Artificial Sequence
  Synthetic Polypeptide
QVQLVQSGAEVKKPGASVKVSCKASGYTFTNYYIHWVRQAPGQRLEYIGWIYPGNVYIQYNEKFKGRATLTADKSASTAYMELSSLRSEDTAVYYCARDGYWFAYWGQGTLVTVSSASTKGPSVFPLAPSSKSTSGGTAALGCLVKDYFPEPVTVSWNSGALTSGVHTFPAVLQSSGLYSLSSVVTVPSSSLGTQTYICNVNHKPSNTKVDKKVEPKSCDKTHTCPPCPAPELLGGPSVFLFPPKPKDTLMISRTPEVTCVVVDVSHEDPEVKFNWYVDGVEVHNAKTKPREEQYNSTYRVVSVLTVLHQDWLNGKEYKCKVSNKALPAPIEKTISKAKGQPREPQVYTLPPSRDELTKNQVSLTCLVKGFYPSDIAVEWESNGQPENNYKTTPPVLDSDGSFFLYSKLTVDKSRWQQGNVFSCSVMHEALHNHYTQKSLSLSPG

SEQ ID NO: 128 - protein, 445 aa, Artificial Sequence
  Synthetic Polypeptide
QVQLVQSGAEVKKPGASVKVSCKASGYTFTNYYIHWVRQAPGQRLEYIGWIYPGNVYIQYNEKFKGRATLTADKSASTAYMELSSLRSEDTAVYYCARDGSWFAYWGQGTLVTVSSASTKGPSVFPLAPSSKSTSGGTAALGCLVKDYFPEPVTVSWNSGALTSGVHTFPAVLQSSGLYSLSSVVTVPSSSLGTQTYICNVNHKPSNTKVDKKVEPKSCDKTHTCPPCPAPELLGGPSVFLFPPKPKDTLMISRTPEVTCVVVDVSHEDPEVKFNWYVDGVEVHNAKTKPREEQYNSTYRVVSVLTVLHQDWLNGKEYKCKVSNKALPAPIEKTISKAKGQPREPQVYTLPPSRDELTKNQVSLTCLVKGFYPSDIAVEWESNGQPENNYKTTPPVLDSDGSFFLYSKLTVDKSRWQQGNVFSCSVMHEALHNHYTQKSLSLSPG

SEQ ID NO: 129 - protein, 445 aa, Artificial Sequence
  Synthetic Polypeptide
QVQLVQSGAEVKKPGASVKVSCKASGYTFTNYYIHWVRQAPGQRLEYIGWIYPGNVYIQYNEKFKGRATLTADKSASTAYMELSSLRSEDTAVYYCARDGFWFAYWGQGTLVTVSSASTKGPSVFPLAPSSKSTSGGTAALGCLVKDYFPEPVTVSWNSGALTSGVHTFPAVLQSSGLYSLSSVVTVPSSSLGTQTYICNVNHKPSNTKVDKKVEPKSCDKTHTCPPCPAPELLGGPSVFLFPPKPKDTLMISRTPEVTCVVVDVSHEDPEVKFNWYVDGVEVHNAKTKPREEQYNSTYRVVSVLTVLHQDWLNGKEYKCKVSNKALPAPIEKTISKAKGQPREPQVYTLPPSRDELTKNQVSLTCLVKGFYPSDIAVEWESNGQPENNYKTTPPVLDSDGSFFLYSKLTVDKSRWQQGNVFSCSVMHEALHNHYTQKSLSLSPG

SEQ ID NO: 130 - protein, 445 aa, Artificial Sequence
  Synthetic Polypeptide
QVQLVQSGAEVKKPGASVKVSCKASGYTFTNYYIHWVRQAPGQRLEYIGWIYPGNVYIQYNEKFKGRATLTADKSASTAYMELSSLRSEDTAVYYCARDGGWFAYWGQGTLVTVSSASTKGPSVFPLAPSSKSTSGGTAALGCLVKDYFPEPVTVSWNSGALTSGVHTFPAVLQSSGLYSLSSVVTVPSSSLGTQTYICNVNHKPSNTKVDKKVEPKSCDKTHTCPPCPAPELLGGPSVFLFPPKPKDTLMISRTPEVTCVVVDVSHEDPEVKFNWYVDGVEVHNAKTKPREEQYNSTYRVVSVLTVLHQDWLNGKEYKCKVSNKALPAPIEKTISKAKGQPREPQVYTLPPSRDELTKNQVSLTCLVKGFYPSDIAVEWESNGQPENNYKTTPPVLDSDGSFFLYSKLTVDKSRWQQGNVFSCSVMHEALHNHYTQKSLSLSPG

SEQ ID NO: 131 - protein, 445 aa, Artificial Sequence
  Synthetic Polypeptide
QVQLVQSGAEVKKPGASVKVSCKASGYTFTNYYIHWVRQAPGQRLEYIGWIYPGNVYIQYNEKFKGRATLTADKSASTAYMELSSLRSEDTAVYYCARDGTWFAYWGQGTLVTVSSASTKGPSVFPLAPSSKSTSGGTAALGCLVKDYFPEPVTVSWNSGALTSGVHTFPAVLQSSGLYSLSSVVTVPSSSLGTQTYICNVNHKPSNTKVDKKVEPKSCDKTHTCPPCPAPELLGGPSVFLFPPKPKDTLMISRTPEVTCVVVDVSHEDPEVKFNWYVDGVEVHNAKTKPREEQYNSTYRVVSVLTVLHQDWLNGKEYKCKVSNKALPAPIEKTISKAKGQPREPQVYTLPPSRDELTKNQVSLTCLVKGFYPSDIAVEWESNGQPENNYKTTPPVLDSDGSFFLYSKLTVDKSRWQQGNVFSCSVMHEALHNHYTQKSLSLSPG

SEQ ID NO: 132 - protein, 445 aa, Artificial Sequence
  Synthetic Polypeptide
QVQLVQSGAEVKKPGASVKVSCKASGYTFTNYYIHWVRQAPGQRLEYIGWIYPGNVYIQYNEKFKGRATLTADKSASTAYMELSSLRSEDTAVYYCARDGVWFAYWGQGTLVTVSSASTKGPSVFPLAPSSKSTSGGTAALGCLVKDYFPEPVTVSWNSGALTSGVHTFPAVLQSSGLYSLSSVVTVPSSSLGTQTYICNVNHKPSNTKVDKKVEPKSCDKTHTCPPCPAPELLGGPSVFLFPPKPKDTLMISRTPEVTCVVVDVSHEDPEVKFNWYVDGVEVHNAKTKPREEQYNSTYRVVSVLTVLHQDWLNGKEYKCKVSNKALPAPIEKTISKAKGQPREPQVYTLPPSRDELTKNQVSLTCLVKGFYPSDIAVEWESNGQPENNYKTTPPVLDSDGSFFLYSKLTVDKSRWQQGNVFSCSVMHEALHNHYTQKSLSLSPG

SEQ ID NO: 133 - protein, 445 aa, Artificial Sequence
  Synthetic Polypeptide
QVQLVQSGAEVKKPGASVKVSCKASGYTFTNYIIHWVRQAPGQRLEYIGWIYPGNVYIQYNEKFKGRATLTADKSASTAYMELSSLRSEDTAVYYCARDGPWFAYWGQGTLVTVSSASTKGPSVFPLAPSSKSTSGGTAALGCLVKDYFPEPVTVSWNSGALTSGVHTFPAVLQSSGLYSLSSVVTVPSSSLGTQTYICNVNHKPSNTKVDKKVEPKSCDKTHTCPPCPAPELLGGPSVFLFPPKPKDTLMISRTPEVTCVVVDVSHEDPEVKFNWYVDGVEVHNAKTKPREEQYNSTYRVVSVLTVLHQDWLNGKEYKCKVSNKALPAPIEKTISKAKGQPREPQVYTLPPSRDELTKNQVSLTCLVKGFYPSDIAVEWESNGQPENNYKTTPPVLDSDGSFFLYSKLTVDKSRWQQGNVFSCSVMHEALHNHYTQKSLSLSPG

SEQ ID NO: 134 - protein, 445 aa, Artificial Sequence
  Synthetic Polypeptide
QVQLVQSGAEVKKPGASVKVSCKASGYTFTNYLIHWVRQAPGQRLEYIGWIYPGNVYIQYNEKFKGRATLTADKSASTAYMELSSLRSEDTAVYYCARDGPWFAYWGQGTLVTVSSASTKGPSVFPLAPSSKSTSGGTAALGCLVKDYFPEPVTVSWNSGALTSGVHTFPAVLQSSGLYSLSSVVTVPSSSLGTQTYICNVNHKPSNTKVDKKVEPKSCDKTHTCPPCPAPELLGGPSVFLFPPKPKDTLMISRTPEVTCVVVDVSHEDPEVKFNWYVDGVEVHNAKTKPREEQYNSTYRVVSVLTVLHQDWLNGKEYKCKVSNKALPAPIEKTISKAKGQPREPQVYTLPPSRDELTKNQVSLTCLVKGFYPSDIAVEWESNGQPENNYKTTPPVLDSDGSFFLYSKLTVDKSRWQQGNVFSCSVMHEALHNHYTQKSLSLSPG

SEQ ID NO: 135 - protein, 219 aa, Artificial Sequence
  Synthetic Polypeptide
DIVLTQTPFSNPVTLGTSASISCRSSKSLLHSDGFTYLYWFLQKPGQSPHLLIYQTSNLASGVPDRFSSSGSGTDFTLRISRVEAEDVGVYYCAQNLELPNTFGGGTKLEIKRADAAPTVSIFPPSSEQLTSGGASVVCFLNNFYPKDINVKWKIDGSERQNGVLNSWTDQDSKDSTYSMSSTLTLTKDEYERHNSYTCEATHKTSTSPIVKSFNRNEC

SEQ ID NO: 136 - protein, 219 aa, Artificial Sequence
  Synthetic Polypeptide
DIVLTQTPFSNPVTLGTSASISCRSSKSLLHSDGFTYLYWFLQKPGQSPHLLIYQTSNLASGVPDRFSSSGSGTDFTLRISRVEAEDVGVYYCAQNLELPNTFGGGTKLEIKRTVAAPSVFIFPPSDEQLKSGTASVVCLLNNFYPREAKVQWKVDNALQSGNSQESVTEQDSKDSTYSLSSTLTLSKADYEKHKVYACEVTHQGLSSPVTKSFNRGEC

SEQ ID NO: 137 - protein, 219 aa, Artificial Sequence
  Synthetic Polypeptide
DIVMTQTPLSLSVTPGQPASISCRSSRSLLHSDGFTYLYWYLQKPGQSPQLLIYQTSNLASGVPDRFSGSGSGTDFTLKISRVEAEDVGVYYCAQNLELPNTFGQGTKLEIKRTVAAPSVFIFPPSDEQLKSGTASVVCLLNNFYPREAKVQWKVDNALQSGNSQESVTEQDSKDSTYSLSSTLTLSKADYEKHKVYACEVTHQGLSSPVTKSFNRGEC

SEQ ID NO: 138 - protein, 219 aa, Artificial Sequence
  Synthetic Polypeptide
DIVLTQTPLSLSVTPGQPASISCRSSKSLLHSDGFTYLYWFLQKPGQSPQLLIYQTSNLASGVPDRFSSSGSGTDFTLKISRVEAEDVGVYYCAQNLELPNTFGQGTKLEIKRTVAAPSVFIFPPSDEQLKSGTASVVCLLNNFYPREAKVQWKVDNALQSGNSQESVTEQDSKDSTYSLSSTLTLSKADYEKHKVYACEVTHQGLSSPVTKSFNRGEC

SEQ ID NO: 139 - protein, 219 aa, Artificial Sequence
  Synthetic Polypeptide
DIVMTQTPLSLSVTPGQPASISCRSSKSLLHSDGFTYLYWFLQKPGQSPQLLIYQTSNLASGVPDRFSGSGSGTDFTLKISRVEAEDVGVYYCAQNLELPNTFGQGTKLEIKRTVAAPSVFIFPPSDEQLKSGTASVVCLLNNFYPREAKVQWKVDNALQSGNSQESVTEQDSKDSTYSLSSTLTLSKADYEKHKVYACEVTHQGLSSPVTKSFNRGEC

SEQ ID NO: 140 - protein, 219 aa, Artificial Sequence
  Synthetic Polypeptide
DIVLTQTPLSLSVTPGQPASISCRSSRSLLHSDGFTYLYWFLQKPGQSPQLLIYQTSNLASGVPDRFSSSGSGTDFTLKISRVEAEDVGVYYCAQNLELPNTFGQGTKLEIKRTVAAPSVFIFPPSDEQLKSGTASVVCLLNNFYPREAKVQWKVDNALQSGNSQESVTEQDSKDSTYSLSSTLTLSKADYEKHKVYACEVTHQGLSSPVTKSFNRGEC

SEQ ID NO: 141 - protein, 219 aa, Artificial Sequence
  Synthetic Polypeptide
DIVLTQTPLSLSVTPGQPASISCRSSRSLLHSNGFTYLYWFLQKPGQSPQLLIYQTSNLASGVPDRFSSSGSGTDFTLKISRVEAEDVGVYYCAQNLELPNTFGQGTKLEIKRTVAAPSVFIFPPSDEQLKSGTASVVCLLNNFYPREAKVQWKVDNALQSGNSQESVTEQDSKDSTYSLSSTLTLSKADYEKHKVYACEVTHQGLSSPVTKSFNRGEC

SEQ ID NO: 142 - protein, 219 aa, Artificial Sequence
  Synthetic Polypeptide
DIVLTQTPLSLSVTPGQPASISCRSSRSLLHSDGITYLYWFLQKPGQSPQLLIYQTSNLASGVPDRFSSSGSGTDFTLKISRVEAEDVGVYYCAQNLELPNTFGQGTKLEIKRTVAAPSVFIFPPSDEQLKSGTASVVCLLNNFYPREAKVQWKVDNALQSGNSQESVTEQDSKDSTYSLSSTLTLSKADYEKHKVYACEVTHQGLSSPVTKSFNRGEC

SEQ ID NO: 143 - protein, 219 aa, Artificial Sequence
  Synthetic Polypeptide
DIVLTQTPLSLSVTPGQPASISCRSSRSLLHSDGFTYLYWFLQKPGQSPQLLIYQTSNLASGVPDRFSSSGSGTDFTLKISRVEAEDVGVYYCAQNLELPWTFGQGTKLEIKRTVAAPSVFIFPPSDEQLKSGTASVVCLLNNFYPREAKVQWKVDNALQSGNSQESVTEQDSKDSTYSLSSTLTLSKADYEKHKVYACEVTHQGLSSPVTKSFNRGEC

SEQ ID NO: 144 - protein, 219 aa, Artificial Sequence
  Synthetic Polypeptide
DIVLTQTPLSLSVTPGQPASISCRSSRSLLHSDGFTYLSWFLQKPGQSPQLLIYQTSNLASGVPDRFSSSGSGTDFTLKISRVEAEDVGVYYCAQNLELPNTFGQGTKLEIKRTVAAPSVFIFPPSDEQLKSGTASVVCLLNNFYPREAKVQWKVDNALQSGNSQESVTEQDSKDSTYSLSSTLTLSKADYEKHKVYACEVTHQGLSSPVTKSFNRGEC

SEQ ID NO: 145 - protein, 219 aa, Artificial Sequence
  Synthetic Polypeptide
DIVLTQTPLSLSVTPGQPASISCRSSRSLLHSDGFTYLYWYLQKPGQSPQLLIYQTSNLASGVPDRFSSSGSGTDFTLKISRVEAEDVGVYYCAQNLELPNTFGQGTKLEIKRTVAAPSVFIFPPSDEQLKSGTASVVCLLNNFYPREAKVQWKVDNALQSGNSQESVTEQDSKDSTYSLSSTLTLSKADYEKHKVYACEVTHQGLSSPVTKSFNRGEC

SEQ ID NO: 146 - protein, 219 aa, Artificial Sequence
  Synthetic Polypeptide
DIVLTQTPLSLSVTPGQPASISCRSSRSLLHSDGFTYLYWFLQKPGQSPQLLIYQTSNLASGVPDRFSSSGSGTDFTLKISRVEAEDVGVYYCQQNLELPNTFGQGTKLEIKRTVAAPSVFIFPPSDEQLKSGTASVVCLLNNFYPREAKVQWKVDNALQSGNSQESVTEQDSKDSTYSLSSTLTLSKADYEKHKVYACEVTHQGLSSPVTKSFNRGEC

SEQ ID NO: 147 - protein, 219 aa, Artificial Sequence
  Synthetic Polypeptide
DIVLTQTPLSLSVTPGQPASISCRSSRSLLHSDGFTYLYWFLQKPGQSPQLLIYQTSNLASGVPDRFSSSGSGTDFTLKISRVEAEDVGVYYCLQNLELPNTFGQGTKLEIKRTVAAPSVFIFPPSDEQLKSGTASVVCLLNNFYPREAKVQWKVDNALQSGNSQESVTEQDSKDSTYSLSSTLTLSKADYEKHKVYACEVTHQGLSSPVTKSFNRGEC

SEQ ID NO: 148 - protein, 219 aa, Artificial Sequence
  Synthetic Polypeptide
DIVLTQTPLSLSVTPGQPASISCRSSRSLLHSDGFTYLYWFLQKPGQSPQLLIYQTSNLASGVPDRFSSSGSGTDFTLKISRVEAEDVGVYYCAQYLELPNTFGQGTKLEIKRTVAAPSVFIFPPSDEQLKSGTASVVCLLNNFYPREAKVQWKVDNALQSGNSQESVTEQDSKDSTYSLSSTLTLSKADYEKHKVYACEVTHQGLSSPVTKSFNRGEC

SEQ ID NO: 149 - protein, 219 aa, Artificial Sequence
  Synthetic Polypeptide
DIVLTQTPLSLSVTPGQPASISCRSSRSLLHSDGFTYLYWFLQKPGQSPQLLIYQTSNLASGVPDRFSSSGSGTDFTLKISRVEAEDVGVYYCAQGLELPNTFGQGTKLEIKRTVAAPSVFIFPPSDEQLKSGTASVVCLLNNFYPREAKVQWKVDNALQSGNSQESVTEQDSKDSTYSLSSTLTLSKADYEKHKVYACEVTHQGLSSPVTKSFNRGEC

SEQ ID NO: 150 - protein, 219 aa, Artificial Sequence
  Synthetic Polypeptide
DIVLTQTPLSLSVTPGQPASISCRSSRSLLHSDGFTYLYWFLQKPGQSPQLLIYQTSNLASGVPDRFSSSGSGTDFTLKISRVEAEDVGVYYCAQSLELPNTFGQGTKLEIKRTVAAPSVFIFPPSDEQLKSGTASVVCLLNNFYPREAKVQWKVDNALQSGNSQESVTEQDSKDSTYSLSSTLTLSKADYEKHKVYACEVTHQGLSSPVTKSFNRGEC

SEQ ID NO: 151 - protein, 15 aa, Artificial Sequence
  Synthetic Polypeptide
PLMTCSDYYTCLNNL

SEQ ID NO: 152 - protein, 15 aa, Artificial Sequence
  Synthetic Polypeptide
LSCTHSRYDMHCPHM

SEQ ID NO: 153 - protein, 15 aa, Artificial Sequence
  Synthetic Polypeptide
HYCHSRTDTITHCNA

SEQ ID NO: 154 - protein, 15 aa, Artificial Sequence
  Synthetic Polypeptide
WCPRLFDRPSMGCPT

SEQ ID NO: 155 - protein, 15 aa, Artificial Sequence
  Synthetic Polypeptide
WWPPCQGGAWCEQRI

SEQ ID NO: 156 - protein, 15 aa, Artificial Sequence
  Synthetic Polypeptide
HSGCPRLFDRCSAPA

SEQ ID NO: 157 - protein, 15 aa, Artificial Sequence
  Synthetic Polypeptide
FICPTLYDRPHCMHT

SEQ ID NO: 158 - protein, 15 aa, Artificial Sequence
  Synthetic Polypeptide
SWCHSATDTILPCSN

SEQ ID NO: 159 - protein, 15 aa, Artificial Sequence
  Synthetic Polypeptide
SPACSDRYYQTCVLN

SEQ ID NO: 160 - protein, 15 aa, Artificial Sequence
  Synthetic Polypeptide
MSCVVDRFDRQCPHL

SEQ ID NO: 161 - protein, 15 aa, Artificial Sequence
  Synthetic Polypeptide
TTRCEHYWFTCPLSP

SEQ ID NO: 162 - protein, 15 aa, Artificial Sequence
  Synthetic Polypeptide
DCTGYSPSVLPACRV

SEQ ID NO: 163 - protein, 15 aa, Artificial Sequence
  Synthetic Polypeptide
FCSGYSPSVLPSCLM

SEQ ID NO: 164 - protein, 15 aa, Artificial Sequence
  Synthetic Polypeptide
SKPCSYMHPYCFYNS

SEQ ID NO: 165 - protein, 15 aa, Artificial Sequence
  Synthetic Polypeptide
LTRCTIAHPYCYYNY

SEQ ID NO: 166 - protein, 15 aa, Artificial Sequence
  Synthetic Polypeptide
PNTCMSERRICSLTY

SEQ ID NO: 167 - protein, 15 aa, Artificial Sequence
  Synthetic Polypeptide
PRPHCAILRQCLAAT

SEQ ID NO: 168 - protein, 18 aa, Artificial Sequence
  Synthetic Polypeptide
AVGLLAPPGGLSGRSDNI

SEQ ID NO: 169 - protein, 14 aa, Artificial Sequence
  Synthetic Polypeptide
SISSGLLSGRSDNI

SEQ ID NO: 170 - protein, 269 aa, Artificial Sequence
  Synthetic Polypeptide
QGQSGQGPLMTCSDYYTCLNNLGGGSSGGAVGLLAPPGGLSGRSDNIGGSDIVLTQTPLSLSVTPGQPASISCRSSRSLLHSDGFTYLYWFLQKPGQSPQLLIYQTSNLASGVPDRFSSSGSGTDFTLKISRVEAEDVGVYYCAQNLELPNTFGQGTKLEIKRTVAAPSVFIFPPSDEQLKSGTASVVCLLNNFYPREAKVQWKVDNALQSGNSQESVTEQDSKDSTYSLSSTLTLSKADYEKHKVYACEVTHQGLSSPVTKSFNRGEC

SEQ ID NO: 171 - protein, 269 aa, Artificial Sequence
  Synthetic Polypeptide
QGQSGQGLSCTHSRYDMHCPHMGGGSSGGAVGLLAPPGGLSGRSDNIGGSDIVLTQTPLSLSVTPGQPASISCRSSRSLLHSDGFTYLYWFLQKPGQSPQLLIYQTSNLASGVPDRFSSSGSGTDFTLKISRVEAEDVGVYYCAQNLELPNTFGQGTKLEIKRTVAAPSVFIFPPSDEQLKSGTASVVCLLNNFYPREAKVQWKVDNALQSGNSQESVTEQDSKDSTYSLSSTLTLSKADYEKHKVYACEVTHQGLSSPVTKSFNRGEC

SEQ ID NO: 172 - protein, 269 aa, Artificial Sequence
  Synthetic Polypeptide
QGQSGQGHYCHSRTDTITHCNAGGGSSGGAVGLLAPPGGLSGRSDNIGGSDIVLTQTPLSLSVTPGQPASISCRSSRSLLHSDGFTYLYWFLQKPGQSPQLLIYQTSNLASGVPDRFSSSGSGTDFTLKISRVEAEDVGVYYCAQNLELPNTFGQGTKLEIKRTVAAPSVFIFPPSDEQLKSGTASVVCLLNNFYPREAKVQWKVDNALQSGNSQESVTEQDSKDSTYSLSSTLTLSKADYEKHKVYACEVTHQGLSSPVTKSFNRGEC

SEQ ID NO: 173 - protein, 269 aa, Artificial Sequence
  Synthetic Polypeptide
QGQSGQGWCPRLFDRPSMGCPTGGGSSGGAVGLLAPPGGLSGRSDNIGGSDIVLTQTPLSLSVTPGQPASISCRSSRSLLHSDGFTYLYWFLQKPGQSPQLLIYQTSNLASGVPDRFSSSGSGTDFTLKISRVEAEDVGVYYCAQNLELPNTFGQGTKLEIKRTVAAPSVFIFPPSDEQLKSGTASVVCLLNNFYPREAKVQWKVDNALQSGNSQESVTEQDSKDSTYSLSSTLTLSKADYEKHKVYACEVTHQGLSSPVTKSFNRGEC

SEQ ID NO: 174 - protein, 269 aa, Artificial Sequence
  Synthetic Polypeptide
QGQSGQGWWPPCQGGAWCEQRIGGGSSGGAVGLLAPPGGLSGRSDNIGGSDIVLTQTPLSLSVTPGQPASISCRSSRSLLHSDGFTYLYWFLQKPGQSPQLLIYQTSNLASGVPDRFSSSGSGTDFTLKISRVEAEDVGVYYCAQNLELPNTFGQGTKLEIKRTVAAPSVFIFPPSDEQLKSGTASVVCLLNNFYPREAKVQWKVDNALQSGNSQESVTEQDSKDSTYSLSSTLTLSKADYEKHKVYACEVTHQGLSSPVTKSFNRGEC

SEQ ID NO: 175 - protein, 269 aa, Artificial Sequence
  Synthetic Polypeptide
QGQSGQGHSGCPRLFDRCSAPAGGGSSGGAVGLLAPPGGLSGRSDNIGGSDIVLTQTPLSLSVTPGQPASISCRSSRSLLHSDGFTYLYWFLQKPGQSPQLLIYQTSNLASGVPDRFSSSGSGTDFTLKISRVEAEDVGVYYCAQNLELPNTFGQGTKLEIKRTVAAPSVFIFPPSDEQLKSGTASVVCLLNNFYPREAKVQWKVDNALQSGNSQESVTEQDSKDSTYSLSSTLTLSKADYEKHKVYACEVTHQGLSSPVTKSFNRGEC

SEQ ID NO: 176 - protein, 269 aa, Artificial Sequence
  Synthetic Polypeptide
QGQSGQGFICPTLYDRPHCMHTGGGSSGGAVGLLAPPGGLSGRSDNIGGSDIVLTQTPLSLSVTPGQPASISCRSSRSLLHSDGFTYLYWFLQKPGQSPQLLIYQTSNLASGVPDRFSSSGSGTDFTLKISRVEAEDVGVYYCAQNLELPNTFGQGTKLEIKRTVAAPSVFIFPPSDEQLKSGTASVVCLLNNFYPREAKVQWKVDNALQSGNSQESVTEQDSKDSTYSLSSTLTLSKADYEKHKVYACEVTHQGLSSPVTKSFNRGEC

SEQ ID NO: 177 - protein, 265 aa, Artificial Sequence
  Synthetic Polypeptide
QGQSGQGPLMTCSDYYTCLNNLGGGSSGGSISSGLLSGRSDNIGGSDIVLTQTPLSLSVTPGQPASISCRSSRSLLHSDGFTYLYWFLQKPGQSPQLLIYQTSNLASGVPDRFSSSGSGTDFTLKISRVEAEDVGVYYCAQNLELPNTFGQGTKLEIKRTVAAPSVFIFPPSDEQLKSGTASVVCLLNNFYPREAKVQWKVDNALQSGNSQESVTEQDSKDSTYSLSSTLTLSKADYEKHKVYACEVTHQGLSSPVTKSFNRGEC

SEQ ID NO: 178 - protein, 265 aa, Artificial Sequence
  Synthetic Polypeptide
QGQSGQGWCPRLFDRPSMGCPTGGGSSGGSISSGLLSGRSDNIGGSDIVLTQTPLSLSVTPGQPASISCRSSRSLLHSDGFTYLYWFLQKPGQSPQLLIYQTSNLASGVPDRFSSSGSGTDFTLKISRVEAEDVGVYYCAQNLELPNTFGQGTKLEIKRTVAAPSVFIFPPSDEQLKSGTASVVCLLNNFYPREAKVQWKVDNALQSGNSQESVTEQDSKDSTYSLSSTLTLSKADYEKHKVYACEVTHQGLSSPVTKSFNRGEC

SEQ ID NO: 179 - protein, 265 aa, Artificial Sequence
  Synthetic Polypeptide
QGQSGQGWWPPCQGGAWCEQRIGGGSSGGSISSGLLSGRSDNIGGSDIVLTQTPLSLSVTPGQPASISCRSSRSLLHSDGFTYLYWFLQKPGQSPQLLIYQTSNLASGVPDRFSSSGSGTDFTLKISRVEAEDVGVYYCAQNLELPNTFGQGTKLEIKRTVAAPSVFIFPPSDEQLKSGTASVVCLLNNFYPREAKVQWKVDNALQSGNSQESVTEQDSKDSTYSLSSTLTLSKADYEKHKVYACEVTHQGLSSPVTKSFNRGEC

SEQ ID NO: 180 - protein, 265 aa, Artificial Sequence
  Synthetic Polypeptide
QGQSGQGHSGCPRLFDRCSAPAGGGSSGGSISSGLLSGRSDNIGGSDIVLTQTPLSLSVTPGQPASISCRSSRSLLHSDGFTYLYWFLQKPGQSPQLLIYQTSNLASGVPDRFSSSGSGTDFTLKISRVEAEDVGVYYCAQNLELPNTFGQGTKLEIKRTVAAPSVFIFPPSDEQLKSGTASVVCLLNNFYPREAKVQWKVDNALQSGNSQESVTEQDSKDSTYSLSSTLTLSKADYEKHKVYACEVTHQGLSSPVTKSFNRGEC

SEQ ID NO: 181 - protein, 265 aa, Artificial Sequence
  Synthetic Polypeptide
QGQSGQGSWCHSATDTILPCSNGGGSSGGSISSGLLSGRSDNIGGSDIVLTQTPLSLSVTPGQPASISCRSSRSLLHSDGFTYLYWFLQKPGQSPQLLIYQTSNLASGVPDRFSSSGSGTDFTLKISRVEAEDVGVYYCAQNLELPNTFGQGTKLEIKRTVAAPSVFIFPPSDEQLKSGTASVVCLLNNFYPREAKVQWKVDNALQSGNSQESVTEQDSKDSTYSLSSTLTLSKADYEKHKVYACEVTHQGLSSPVTKSFNRGEC

SEQ ID NO: 182 - protein, 265 aa, Artificial Sequence
  Synthetic Polypeptide
QGQSGQGSPACSDRYYQTCVLNGGGSSGGSISSGLLSGRSDNIGGSDIVLTQTPLSLSVTPGQPASISCRSSRSLLHSDGFTYLYWFLQKPGQSPQLLIYQTSNLASGVPDRFSSSGSGTDFTLKISRVEAEDVGVYYCAQNLELPNTFGQGTKLEIKRTVAAPSVFIFPPSDEQLKSGTASVVCLLNNFYPREAKVQWKVDNALQSGNSQESVTEQDSKDSTYSLSSTLTLSKADYEKHKVYACEVTHQGLSSPVTKSFNRGEC

SEQ ID NO: 183 - protein, 265 aa, Artificial Sequence
  Synthetic Polypeptide
QGQSGQGMSCVVDRFDRQCPHLGGGSSGGSISSGLLSGRSDNIGGSDIVLTQTPLSLSVTPGQPASISCRSSRSLLHSDGFTYLYWFLQKPGQSPQLLIYQTSNLASGVPDRFSSSGSGTDFTLKISRVEAEDVGVYYCAQNLELPNTFGQGTKLEIKRTVAAPSVFIFPPSDEQLKSGTASVVCLLNNFYPREAKVQWKVDNALQSGNSQESVTEQDSKDSTYSLSSTLTLSKADYEKHKVYACEVTHQGLSSPVTKSFNRGEC

SEQ ID NO: 184 - protein, 265 aa, Artificial Sequence
  Synthetic Polypeptide
QGQSGQGTTRCEHYWFTCPLSPGGGSSGGSISSGLLSGRSDNIGGSDIVLTQTPLSLSVTPGQPASISCRSSRSLLHSDGFTYLYWFLQKPGQSPQLLIYQTSNLASGVPDRFSSSGSGTDFTLKISRVEAEDVGVYYCAQNLELPNTFGQGTKLEIKRTVAAPSVFIFPPSDEQLKSGTASVVCLLNNFYPREAKVQWKVDNALQSGNSQESVTEQDSKDSTYSLSSTLTLSKADYEKHKVYACEVTHQGLSSPVTKSFNRGEC

SEQ ID NO: 185 - protein, 269 aa, Artificial Sequence
  Synthetic Polypeptide
QGQSGQGSWCHSATDTILPCSNGGGSSGGAVGLLAPPGGLSGRSDNIGGSDIVLTQTPLSLSVTPGQPASISCRSSRSLLHSDGFTYLYWFLQKPGQSPQLLIYQTSNLASGVPDRFSSSGSGTDFTLKISRVEAEDVGVYYCAQNLELPNTFGQGTKLEIKRTVAAPSVFIFPPSDEQLKSGTASVVCLLNNFYPREAKVQWKVDNALQSGNSQESVTEQDSKDSTYSLSSTLTLSKADYEKHKVYACEVTHQGLSSPVTKSFNRGEC

SEQ ID NO: 186 - protein, 269 aa, Artificial Sequence
  Synthetic Polypeptide
QGQSGQGSPACSDRYYQTCVLNGGGSSGGAVGLLAPPGGLSGRSDNIGGSDIVLTQTPLSLSVTPGQPASISCRSSRSLLHSDGFTYLYWFLQKPGQSPQLLIYQTSNLASGVPDRFSSSGSGTDFTLKISRVEAEDVGVYYCAQNLELPNTFGQGTKLEIKRTVAAPSVFIFPPSDEQLKSGTASVVCLLNNFYPREAKVQWKVDNALQSGNSQESVTEQDSKDSTYSLSSTLTLSKADYEKHKVYACEVTHQGLSSPVTKSFNRGEC

SEQ ID NO: 187 - protein, 269 aa, Artificial Sequence
  Synthetic Polypeptide
QGQSGQGMSCVVDRFDRQCPHLGGGSSGGAVGLLAPPGGLSGRSDNIGGSDIVLTQTPLSLSVTPGQPASISCRSSRSLLHSDGFTYLYWFLQKPGQSPQLLIYQTSNLASGVPDRFSSSGSGTDFTLKISRVEAEDVGVYYCAQNLELPNTFGQGTKLEIKRTVAAPSVFIFPPSDEQLKSGTASVVCLLNNFYPREAKVQWKVDNALQSGNSQESVTEQDSKDSTYSLSSTLTLSKADYEKHKVYACEVTHQGLSSPVTKSFNRGEC

SEQ ID NO: 188 - protein, 269 aa, Artificial Sequence
  Synthetic Polypeptide
QGQSGQGTTRCEHYWFTCPLSPGGGSSGGAVGLLAPPGGLSGRSDNIGGSDIVLTQTPLSLSVTPGQPASISCRSSRSLLHSDGFTYLYWFLQKPGQSPQLLIYQTSNLASGVPDRFSSSGSGTDFTLKISRVEAEDVGVYYCAQNLELPNTFGQGTKLEIKRTVAAPSVFIFPPSDEQLKSGTASVVCLLNNFYPREAKVQWKVDNALQSGNSQESVTEQDSKDSTYSLSSTLTLSKADYEKHKVYACEVTHQGLSSPVTKSFNRGEC

SEQ ID NO: 189 - protein, 265 aa, Artificial Sequence
  Synthetic Polypeptide
QGQSGQGDCTGYSPSVLPACRVGGGSSGGSISSGLLSGRSDNIGGSDIVLTQTPLSLSVTPGQPASISCRSSRSLLHSDGFTYLYWFLQKPGQSPQLLIYQTSNLASGVPDRFSSSGSGTDFTLKISRVEAEDVGVYYCAQNLELPNTFGQGTKLEIKRTVAAPSVFIFPPSDEQLKSGTASVVCLLNNFYPREAKVQWKVDNALQSGNSQESVTEQDSKDSTYSLSSTLTLSKADYEKHKVYACEVTHQGLSSPVTKSFNRGEC

SEQ ID NO: 190 - protein, 265 aa, Artificial Sequence
  Synthetic Polypeptide
QGQSGQGFCSGYSPSVLPSCLMGGGSSGGSISSGLLSGRSDNIGGSDIVLTQTPLSLSVTPGQPASISCRSSRSLLHSDGFTYLYWFLQKPGQSPQLLIYQTSNLASGVPDRFSSSGSGTDFTLKISRVEAEDVGVYYCAQNLELPNTFGQGTKLEIKRTVAAPSVFIFPPSDEQLKSGTASVVCLLNNFYPREAKVQWKVDNALQSGNSQESVTEQDSKDSTYSLSSTLTLSKADYEKHKVYACEVTHQGLSSPVTKSFNRGEC

SEQ ID NO: 191 - protein, 265 aa, Artificial Sequence
  Synthetic Polypeptide
QGQSGQGSKPCSYMHPYCFYNSGGGSSGGSISSGLLSGRSDNIGGSDIVLTQTPLSLSVTPGQPASISCRSSRSLLHSDGFTYLYWFLQKPGQSPQLLIYQTSNLASGVPDRFSSSGSGTDFTLKISRVEAEDVGVYYCAQNLELPNTFGQGTKLEIKRTVAAPSVFIFPPSDEQLKSGTASVVCLLNNFYPREAKVQWKVDNALQSGNSQESVTEQDSKDSTYSLSSTLTLSKADYEKHKVYACEVTHQGLSSPVTKSFNRGEC

SEQ ID NO: 192 - protein, 265 aa, Artificial Sequence
  Synthetic Polypeptide
QGQSGQGLTRCTIAHPYCYYNYGGGSSGGSISSGLLSGRSDNIGGSDIVLTQTPLSLSVTPGQPASISCRSSRSLLHSDGFTYLYWFLQKPGQSPQLLIYQTSNLASGVPDRFSSSGSGTDFTLKISRVEAEDVGVYYCAQNLELPNTFGQGTKLEIKRTVAAPSVFIFPPSDEQLKSGTASVVCLLNNFYPREAKVQWKVDNALQSGNSQESVTEQDSKDSTYSLSSTLTLSKADYEKHKVYACEVTHQGLSSPVTKSFNRGEC

SEQ ID NO: 193 - protein, 265 aa, Artificial Sequence
  Synthetic Polypeptide
QGQSGQGPNTCMSERRICSLTYGGGSSGGSISSGLLSGRSDNIGGSDIVLTQTPLSLSVTPGQPASISCRSSRSLLHSDGFTYLYWFLQKPGQSPQLLIYQTSNLASGVPDRFSSSGSGTDFTLKISRVEAEDVGVYYCAQNLELPNTFGQGTKLEIKRTVAAPSVFIFPPSDEQLKSGTASVVCLLNNFYPREAKVQWKVDNALQSGNSQESVTEQDSKDSTYSLSSTLTLSKADYEKHKVYACEVTHQGLSSPVTKSFNRGEC

SEQ ID NO: 194 - protein, 265 aa, Artificial Sequence
  Synthetic Polypeptide
QGQSGQGPRPHCAILRQCLAATGGGSSGGSISSGLLSGRSDNIGGSDIVLTQTPLSLSVTPGQPASISCRSSRSLLHSDGFTYLYWFLQKPGQSPQLLIYQTSNLASGVPDRFSSSGSGTDFTLKISRVEAEDVGVYYCAQNLELPNTFGQGTKLEIKRTVAAPSVFIFPPSDEQLKSGTASVVCLLNNFYPREAKVQWKVDNALQSGNSQESVTEQDSKDSTYSLSSTLTLSKADYEKHKVYACEVTHQGLSSPVTKSFNRGEC

SEQ ID NO: 195 - protein, 269 aa, Artificial Sequence
  Synthetic Polypeptide
QGQSGQGDCTGYSPSVLPACRVGGGSSGGAVGLLAPPGGLSGRSDNIGGSDIVLTQTPLSLSVTPGQPASISCRSSRSLLHSDGFTYLYWFLQKPGQSPQLLIYQTSNLASGVPDRFSSSGSGTDFTLKISRVEAEDVGVYYCAQNLELPNTFGQGTKLEIKRTVAAPSVFIFPPSDEQLKSGTASVVCLLNNFYPREAKVQWKVDNALQSGNSQESVTEQDSKDSTYSLSSTLTLSKADYEKHKVYACEVTHQGLSSPVTKSFNRGEC

SEQ ID NO: 196 - protein, 269 aa, Artificial Sequence
  Synthetic Polypeptide
QGQSGQGFCSGYSPSVLPSCLMGGGSSGGAVGLLAPPGGLSGRSDNIGGSDIVLTQTPLSLSVTPGQPASISCRSSRSLLHSDGFTYLYWFLQKPGQSPQLLIYQTSNLASGVPDRFSSSGSGTDFTLKISRVEAEDVGVYYCAQNLELPNTFGQGTKLEIKRTVAAPSVFIFPPSDEQLKSGTASVVCLLNNFYPREAKVQWKVDNALQSGNSQESVTEQDSKDSTYSLSSTLTLSKADYEKHKVYACEVTHQGLSSPVTKSFNRGEC

SEQ ID NO: 197 - protein, 269 aa, Artificial Sequence
  Synthetic Polypeptide
QGQSGQGSKPCSYMHPYCFYNSGGGSSGGAVGLLAPPGGLSGRSDNIGGSDIVLTQTPLSLSVTPGQPASISCRSSRSLLHSDGFTYLYWFLQKPGQSPQLLIYQTSNLASGVPDRFSSSGSGTDFTLKISRVEAEDVGVYYCAQNLELPNTFGQGTKLEIKRTVAAPSVFIFPPSDEQLKSGTASVVCLLNNFYPREAKVQWKVDNALQSGNSQESVTEQDSKDSTYSLSSTLTLSKADYEKHKVYACEVTHQGLSSPVTKSFNRGEC

SEQ ID NO: 198 - protein, 269 aa, Artificial Sequence
  Synthetic Polypeptide
QGQSGQGLTRCTIAHPYCYYNYGGGSSGGAVGLLAPPGGLSGRSDNIGGSDIVLTQTPLSLSVTPGQPASISCRSSRSLLHSDGFTYLYWFLQKPGQSPQLLIYQTSNLASGVPDRFSSSGSGTDFTLKISRVEAEDVGVYYCAQNLELPNTFGQGTKLEIKRTVAAPSVFIFPPSDEQLKSGTASVVCLLNNFYPREAKVQWKVDNALQSGNSQESVTEQDSKDSTYSLSSTLTLSKADYEKHKVYACEVTHQGLSSPVTKSFNRGEC

SEQ ID NO: 199 - protein, 269 aa, Artificial Sequence
  Synthetic Polypeptide
QGQSGQGPNTCMSERRICSLTYGGGSSGGAVGLLAPPGGLSGRSDNIGGSDIVLTQTPLSLSVTPGQPASISCRSSRSLLHSDGFTYLYWFLQKPGQSPQLLIYQTSNLASGVPDRFSSSGSGTDFTLKISRVEAEDVGVYYCAQNLELPNTFGQGTKLEIKRTVAAPSVFIFPPSDEQLKSGTASVVCLLNNFYPREAKVQWKVDNALQSGNSQESVTEQDSKDSTYSLSSTLTLSKADYEKHKVYACEVTHQGLSSPVTKSFNRGEC

SEQ ID NO: 200 - protein, 269 aa, Artificial Sequence
  Synthetic Polypeptide
QGQSGQGPRPHCAILRQCLAATGGGSSGGAVGLLAPPGGLSGRSDNIGGSDIVLTQTPLSLSVTPGQPASISCRSSRSLLHSDGFTYLYWFLQKPGQSPQLLIYQTSNLASGVPDRFSSSGSGTDFTLKISRVEAEDVGVYYCAQNLELPNTFGQGTKLEIKRTVAAPSVFIFPPSDEQLKSGTASVVCLLNNFYPREAKVQWKVDNALQSGNSQESVTEQDSKDSTYSLSSTLTLSKADYEKHKVYACEVTHQGLSSPVTKSFNRGEC

SEQ ID NO: 201 - DNA, 1335 bp, Artificial Sequence
  Synthetic Oligonucleotide
gaggtgaagctggaggagagcggccccgccctggtgaagcctggagcttccgtgaggatcagctgtaaggcctctggctacacctttacaaactactatatccattgggtgaagcagcggccaggacagggcctggactacatcggctggatctatcccggcaacgtgtacatccagtataatgagaagttcaagggcaaggccaccctgacagctgataagtccagctctaccgcttttatgcagctgtccagcctgacaagcgaggactctgccgtgtacttctgcgctagggatggcccttggtttgcctattggggccagggcaccctggtgacagtgtcttccgcttccaccaagggcccatcagttttccccttggctccaagttctaaatccacaagcggtggaacagctgcactgggatgcctcgttaaagattatttccctgagcctgtgacagtgagctggaatagcggagcattgacttcaggtgtgcacacttttcccgctgtgttgcagtcctccggtctgtactcactgtccagtgtcgtaaccgtcccttctagcagcttgggaacccagacctacatctgtaacgtcaaccataaaccatccaacacaaaggtggataagaaggttgaaccaaagagctgtgataagacacatacatgccctccttgtcctgcaccagagctcctcggaggtccatctgtgttcctgtttccccccaaacccaaggacactcttatgatctctcgtactccagaggtcacctgtgttgttgtcgacgtgagccatgaagatcccgaggttaaattcaactggtacgtggatggagtcgaggttcacaatgccaagaccaagcccagggaggagcaatataattctacatatcgggtagtgagcgttctgaccgtgctccaccaagattggctcaatggaaaagagtacaagtgcaaggtgtccaacaaggctcttcccgctcccattgagaaaactatctccaaagccaaggggcagccacgggaaccccaggtgtatacattgcccccatctagagacgagctgaccaagaaccaggtgagtctcacttgtctggtcaaggggttttacccttctgacattgctgtagagtgggagtctaacggacagccagaaaacaactacaagacaactcccccagtgctggacagcgacgggagcttcttcctctactccaagttgactgtagacaagtctagatggcagcaaggaaacgttttctcctgctcagtaatgcatgaggctctgcacaatcactatacccagaaatcactgtcccttagcccaggg

SEQ ID NO: 202 - DNA, 657 bp, Artificial Sequence
  Synthetic Oligonucleotide
gatattgtgctgacccagactccattctccaatcccgtcactcttggaacatcagcttccatctcctgcaggtctagtaagagtctcctacatagtgatggcttcacttatttgtattggtttctgcagaagccaggccagtctcctcatctcctgatttatcagacgtccaaccttgcctcaggagtcccagacaggttcagtagcagtgggtcaggaactgatttcacactgagaatcagcagagtggaggctgaagatgtgggtgtttattactgtgctcaaaatctagaacttcccaacacgttcggaggggggaccaagctggaaatcaaacgtacggtggctgcaccatctgtcttcatcttcccgccatctgatgagcagttgaaatctggaactgcctctgttgtgtgcctgctgaataacttctatcccagagaggccaaagtacagtggaaggtggataacgccctccaatcgggtaactcccaggagagtgtcacagagcaggacagcaaggacagcacctacagcctcagcagcaccctgacgctgagcaaagcagactacgagaaacacaaagtctacgcctgcgaagtcacccatcagggcctgagctcgcccgtcacaaagagcttcaacaggggagagtgt

SEQ ID NO: 203 - DNA, 1335 bp, Artificial Sequence
  Synthetic Oligonucleotide
caggtgcagctggtgcagagcggagctgaggtgaagaagccaggagcttccgtgaaggtgagctgtaaggcctctggctacaccttcacaaactactatatccattgggtgaggcaggctccaggacagcggctggagtacatcggatggatctatcctggcaacgtgtacatccagtataatgagaagtttaagggcagggccaccctgacagctgacaagagcgcctctaccgcttacatggagctgtccagcctgagatctgaggacacagccgtgtactattgcgctcgcgatggcccttggtttgcctattggggccagggcaccctggtgacagtgtcttccgcttccaccaagggcccatcagttttccccttggctccaagttctaaatccacaagcggtggaacagctgcactgggatgcctcgttaaagattatttccctgagcctgtgacagtgagctggaatagcggagcattgacttcaggtgtgcacacttttcccgctgtgttgcagtcctccggtctgtactcactgtccagtgtcgtaaccgtcccttctagcagcttgggaacccagacctacatctgtaacgtcaaccataaaccatccaacacaaaggtggataagaaggttgaaccaaagagctgtgataagacacatacatgccctccttgtcctgcaccagagctcctcggaggtccatctgtgttcctgtttccccccaaacccaaggacactcttatgatctctcgtactccagaggtcacctgtgttgttgtcgacgtgagccatgaagatcccgaggttaaattcaactggtacgtggatggagtcgaggttcacaatgccaagaccaagcccagggaggagcaatataattctacatatcgggtagtgagcgttctgaccgtgctccaccaagattggctcaatggaaaagagtacaagtgcaaggtgtccaacaaggctcttcccgctcccattgagaaaactatctccaaagccaaggggcagccacgggaaccccaggtgtatacattgcccccatctagagacgagctgaccaagaaccaggtgagtctcacttgtctggtcaaggggttttacccttctgacattgctgtagagtgggagtctaacggacagccagaaaacaactacaagacaactcccccagtgctggacagcgacgggagcttcttcctctactccaagttgactgtagacaagtctagatggcagcaaggaaacgttttctcctgctcagtaatgcatgaggctctgcacaatcactatacccagaaatcactgtcccttagcccaggg

SEQ ID NO: 204 - DNA, 657 bp, Artificial Sequence
  Synthetic Oligonucleotide
gacatcgtgctgacccagacaccactgtctctgtccgtgaccccaggacagcctgctagcatctcttgtaggtccagcaggtccctgctgcatagcgatggcttcacctacctgtattggtttctgcagaagccaggccagtctccccagctgctgatctaccagacatctaacctggcttccggcgtgcctgacaggttctcttccagcggcagcggcaccgacttcaccctgaagatctctcgggtggaggctgaggacgtgggcgtgtactattgcgctcagaacctggagctgccaaatacctttggccagggcacaaagctggagatcaagcgtacggtggctgcaccatctgtcttcatcttcccgccatctgatgagcagttgaaatctggaactgcctctgttgtgtgcctgctgaataacttctatcccagagaggccaaagtacagtggaaggtggataacgccctccaatcgggtaactcccaggagagtgtcacagagcaggacagcaaggacagcacctacagcctcagcagcaccctgacgctgagcaaagcagactacgagaaacacaaagtctacgcctgcgaagtcacccatcagggcctgagctcgcccgtcacaaagagcttcaacaggggagagtgt

SEQ ID NO: 205 - DNA, 1338 bp, Artificial Sequence
  Synthetic Oligonucleotide
caggtgcagctggtgcagagcggagctgaggtgaagaagccaggagcttccgtgaaggtgagctgtaaggcctctggctacaccttcacaaactaccacatccattgggtgaggcaggctccaggacagcggctggagtacatcggatggatctatcctggcaacgtgtacatccagtataatgagaagtttaagggcagggccaccctgacagctgacaagagcgcctctaccgcttacatggagctgtccagcctgagatctgaggacacagccgtgtactattgcgctcgcgatggcccttggtttgcctattggggccagggcaccctggtgacagtgtcttccgcttccaccaagggcccatcagttttccccttggctccaagttctaaatccacaagcggtggaacagctgcactgggatgcctcgttaaagattatttccctgagcctgtgacagtgagctggaatagcggagcattgacttcaggtgtgcacacttttcccgctgtgttgcagtcctccggtctgtactcactgtccagtgtcgtaaccgtcccttctagcagcttgggaacccagacctacatctgtaacgtcaaccataaaccatccaacacaaaggtggataagaaggttgaaccaaagagctgtgataagacacatacatgccctccttgtcctgcaccagagctcctcggaggtccatctgtgttcctgtttccccccaaacccaaggacactcttatgatctctcgtactccagaggtcacctgtgttgttgtcgacgtgagccatgaagatcccgaggttaaattcaactggtacgtggatggagtcgaggttcacaatgccaagaccaagcccagggaggagcaatataattctacatatcgggtagtgagcgttctgaccgtgctccaccaagattggctcaatggaaaagagtacaagtgcaaggtgtccaacaaggctcttcccgctcccattgagaaaactatctccaaagccaaggggcagccacgggaaccccaggtgtatacattgcccccatctagagacgagctgaccaagaaccaggtgagtctcacttgtctggtcaaggggttttacccttctgacattgctgtagagtgggagtctaacggacagccagaaaacaactacaagacaactcccccagtgctggacagcgacgggagcttcttcctctactccaagttgactgtagacaagtctagatggcagcaaggaaacgttttctcctgctcagtaatgcatgaggctctgcacaatcactatacccagaaatcactgtcccttagcccagggtga

SEQ ID NO: 206 - DNA, 1338 bp, Artificial Sequence
  Synthetic Oligonucleotide
caggtgcagctggtgcagagcggagctgaggtgaagaagccaggagcttccgtgaaggtgagctgtaaggcctctggctacaccttcacaaactacgacatccattgggtgaggcaggctccaggacagcggctggagtacatcggatggatctatcctggcaacgtgtacatccagtataatgagaagtttaagggcagggccaccctgacagctgacaagagcgcctctaccgcttacatggagctgtccagcctgagatctgaggacacagccgtgtactattgcgctcgcgatggcccttggtttgcctattggggccagggcaccctggtgacagtgtcttccgcttccaccaagggcccatcagttttccccttggctccaagttctaaatccacaagcggtggaacagctgcactgggatgcctcgttaaagattatttccctgagcctgtgacagtgagctggaatagcggagcattgacttcaggtgtgcacacttttcccgctgtgttgcagtcctccggtctgtactcactgtccagtgtcgtaaccgtcccttctagcagcttgggaacccagacctacatctgtaacgtcaaccataaaccatccaacacaaaggtggataagaaggttgaaccaaagagctgtgataagacacatacatgccctccttgtcctgcaccagagctcctcggaggtccatctgtgttcctgtttccccccaaacccaaggacactcttatgatctctcgtactccagaggtcacctgtgttgttgtcgacgtgagccatgaagatcccgaggttaaattcaactggtacgtggatggagtcgaggttcacaatgccaagaccaagcccagggaggagcaatataattctacatatcgggtagtgagcgttctgaccgtgctccaccaagattggctcaatggaaaagagtacaagtgcaaggtgtccaacaaggctcttcccgctcccattgagaaaactatctccaaagccaaggggcagccacgggaaccccaggtgtatacattgcccccatctagagacgagctgaccaagaaccaggtgagtctcacttgtctggtcaaggggttttacccttctgacattgctgtagagtgggagtctaacggacagccagaaaacaactacaagacaactcccccagtgctggacagcgacgggagcttcttcctctactccaagttgactgtagacaagtctagatggcagcaaggaaacgttttctcctgctcagtaatgcatgaggctctgcacaatcactatacccagaaatcactgtcccttagcccagggtga

SEQ ID NO: 207 - DNA, 1338 bp, Artificial Sequence
  Synthetic Oligonucleotide
caggtgcagctggtgcagagcggagctgaggtgaagaagccaggagcttccgtgaaggtgagctgtaaggcctctggctacaccttcacaaactactatatccattgggtgaggcaggctccaggacagcggctggagtacatcggatggatctatcctggcaacgtgtacatccagtataatgagaagtttaagggcagggccaccctgacagctgacaagagcgcctctaccgcttacatggagctgtccagcctgagatctgaggacacagccgtgtactattgcgctcgcgatggctactggtttgcctattggggccagggcaccctggtgacagtgtcttccgcttccaccaagggcccatcagttttccccttggctccaagttctaaatccacaagcggtggaacagctgcactgggatgcctcgttaaagattatttccctgagcctgtgacagtgagctggaatagcggagcattgacttcaggtgtgcacacttttcccgctgtgttgcagtcctccggtctgtactcactgtccagtgtcgtaaccgtcccttctagcagcttgggaacccagacctacatctgtaacgtcaaccataaaccatccaacacaaaggtggataagaaggttgaaccaaagagctgtgataagacacatacatgccctccttgtcctgcaccagagctcctcggaggtccatctgtgttcctgtttccccccaaacccaaggacactcttatgatctctcgtactccagaggtcacctgtgttgttgtcgacgtgagccatgaagatcccgaggttaaattcaactggtacgtggatggagtcgaggttcacaatgccaagaccaagcccagggaggagcaatataattctacatatcgggtagtgagcgttctgaccgtgctccaccaagattggctcaatggaaaagagtacaagtgcaaggtgtccaacaaggctcttcccgctcccattgagaaaactatctccaaagccaaggggcagccacgggaaccccaggtgtatacattgcccccatctagagacgagctgaccaagaaccaggtgagtctcacttgtctggtcaaggggttttacccttctgacattgctgtagagtgggagtctaacggacagccagaaaacaactacaagacaactcccccagtgctggacagcgacgggagcttcttcctctactccaagttgactgtagacaagtctagatggcagcaaggaaacgttttctcctgctcagtaatgcatgaggctctgcacaatcactatacccagaaatcactgtcccttagcccagggtga

SEQ ID NO: 208 - DNA, 807 bp, Artificial Sequence
  Synthetic Oligonucleotide
cagggacagtctggacagggatggtggccaccttgccagggaggagcttggtgtgagcagaggatcggaggaggctccagcggaggagctgtgggcctgctggctccaccaggaggactgtctggcagatccgacaacatcggcggctccgatatcgtgctgacccagacacccctgagcctgtctgtgacccctggccagccagcctccatcagctgcaggtcttcccggtccctgctgcatagcgacggcttcacctacctgtattggtttctgcagaagcccggccagagccctcagctgctgatctaccagacatctaatctggcttccggcgtgccagacagattcagctcttccggcagcggcaccgacttcaccctgaagatctctcgcgtggaggccgaggatgtgggcgtgtactattgtgctcagaacctggagctgcccaatacctttggccagggcacaaagctggagatcaagcgtacggtggctgcaccatctgtcttcatcttcccgccatctgatgagcagttgaaatctggaactgcctctgttgtgtgcctgctgaataacttctatcccagagaggccaaagtacagtggaaggtggataacgccctccaatcgggtaactcccaggagagtgtcacagagcaggacagcaaggacagcacctacagcctcagcagcaccctgacgctgagcaaagcagactacgagaaacacaaagtctacgcctgcgaagtcacccatcagggcctgagctcgcccgtcacaaagagcttcaacaggggagagtgt

SEQ ID NO: 209 - DNA, 795 bp, Artificial Sequence
  Synthetic Oligonucleotide
cagggacagagcggacagggatggtggccaccttgccagggaggagcttggtgtgagcagaggatcggaggaggctccagcggaggctctatctcttccggcctgctgagcggcagatctgacaacatcggcggctccgatatcgtgctgacccagacaccactgtccctgagcgtgaccccaggacagccagcctctatctcctgcaggagctctcggtctctgctgcattccgacggcttcacctacctgtattggtttctgcagaagcctggccagtctccacagctgctgatctaccagacaagcaatctggcttctggcgtgcccgacagattctccagctctggctccggcaccgacttcaccctgaagatcagccgcgtggaggctgaggatgtgggcgtgtactattgtgctcagaacctggagctgcctaatacctttggccagggcacaaagctggagatcaagcgtacggtggctgcaccatctgtcttcatcttcccgccatctgatgagcagttgaaatctggaactgcctctgttgtgtgcctgctgaataacttctatcccagagaggccaaagtacagtggaaggtggataacgccctccaatcgggtaactcccaggagagtgtcacagagcaggacagcaaggacagcacctacagcctcagcagcaccctgacgctgagcaaagcagactacgagaaacacaaagtctacgcctgcgaagtcacccatcagggcctgagctcgcccgtcacaaagagcttcaacaggggagagtgt

SEQ ID NO: 210 - protein, 283 aa, Artificial Sequence
  Synthetic Polypeptide
QRDCVCDNYKLATSCSLNEYGECQCTSYGTQNTVICSKLASKCLAMKAEMTHSKSGRRIKPEGAIQNNDGLYDPDCDEQGSKCLAMKAEMTHSKSGRRIKPEGAIQNNDGLYDPDCDEQGLFKAKQCNGTATCWCVNTAGVRRTDKDTEITCSERVRTYWIIIELKHKERESPYDHQSLQTALQEAFTSRYKLNQKFIKNIMYENNVITIDLMQNSSQKTQDDVDIADVAYYFEKDVKGESLFHSSKSMDLRVNGEPLDLDPGQTLIYYVDEKAPEFSMQGLT

SEQ ID NO: 211 - protein, 282 aa, Artificial Sequence
  Synthetic Polypeptide
QRDCVCDNYKLATSCSLNEYGECQCTSYGTQNTVICSKLAAKCLVMKAEMNGSKLGRRAKPEGALQNNDGLYDPDCDESGAKCLVMKAEMNGSKLGRRAKPEGALQNNDGLYDPDCDESGLFKAKQCNGTSMCWCVNTAGVRRTDKDTEITCSERVRTYWIIIELKHKAREKPYDSKSLRTALQKEITTRYQLDPKFITSILYENNVITIDLVQNSSQKTQNDVDIADVAYYFEKDVKGESLFHSKKMDLTVNGEQLDLDPGQTLIYYVDEKAPEFSMQGLK

SEQ ID NO: 212 - protein, 282 aa, Artificial Sequence
  Synthetic Polypeptide
QEECVCENYKLAVNCFVNNNRQCQCTSVGAQNTVICSKLAAKCLAMKAEMTHSKSGRRIKPEGAIQNNDGLYDPDCDEQGAKCLAMKAEMTHSKSGRRIKPEGAIQNNDGLYDPDCDEQGLFKAKQCNGTATCWCVNTAGVRRTDKDTEITCSERVRTYWIIIELKHKAREKPYDSKSLRTALQKEITTRYQLDPKFITSILYENNVITIDLVQNSSQKTQNDVDIADVAYYFEKDVKGESLFHSKKMDLTVNGEQLDLDPGQTLIYYVDEKAPEFSMQGLK

SEQ ID NO: 213 - protein, 282 aa, Artificial Sequence
  Synthetic Polypeptide
QRDCVCDNYKLATSCSLNEYGECQCTSYGTQNTVICSKLASKCLAMKAEMTHSKSGRRIKPEGAIQNNDGLYDPDCDEQGSKCLAMKAEMTHSKSGRRIKPEGAIQNNDGLYDPDCDEQGLFKAKQCNGTATCWCVNTAGVRRTDKDTEITCSERVRTYWIIIELKHKAREKPYDSKSLRTALQKEITTRYQLDPKFITSILYENNVITIDLVQNSSQKTQNDVDIADVAYYFEKDVKGESLFHSKKMDLTVNGEQLDLDPGQTLIYYVDEKAPEFSMQGLK

SEQ ID NO: 214 - protein, 283 aa, Artificial Sequence
  Synthetic Polypeptide
QEECVCENYKLAVNCFVNNNRQCQCTSVGAQNTVICSKLAAKCLVMKAEMNGSKLGRRAKPEGALQNNDGLYDPDCDESGAKCLVMKAEMNGSKLGRRAKPEGALQNNDGLYDPDCDESGLFKAKQCNGTSMCWCVNTAGVRRTDKDTEITCSERVRTYWIIIELKHKERESPYDHQSLQTALQEAFTSRYKLNQKFIKNIMYENNVITIDLMQNSSQKTQDDVDIADVAYYFEKDVKGESLFHSSKSMDLRVNGEPLDLDPGQTLIYYVDEKAPEFSMQGLT

SEQ ID NO: 215 - protein, 4 aa, Artificial Sequence
  Synthetic Polypeptide
ALAL

SEQ ID NO: 216 - protein, 4 aa, Artificial Sequence
  Synthetic Polypeptide
ALAL

SEQ ID NO: 217 - protein, 4 aa, Artificial Sequence
  Synthetic Polypeptide
GFLG

SEQ ID NO: 218 - protein, 15 aa, Artificial Sequence
  Synthetic Polypeptide
PLMTCSDYYTCKNNL

SEQ ID NO: 219 - protein, 15 aa, Artificial Sequence
  Synthetic Polypeptide
PLMTCSDYYTCHNNL

SEQ ID NO: 220 - protein, 15 aa, Artificial Sequence
  Synthetic Polypeptide
PLMTCSDYYTCRNNL

SEQ ID NO: 221 - protein, 15 aa, Artificial Sequence
  Synthetic Polypeptide
KFSCTTMPHKNCMKP

SEQ ID NO: 222 - protein, 15 aa, Artificial Sequence
  Synthetic Polypeptide
PLMTCTKYNNCINNL

SEQ ID NO: 223 - protein, 15 aa, Artificial Sequence
  Synthetic Polypeptide
PNYMCKLNTCTHHIA

SEQ ID NO: 224 - protein, 15 aa, Artificial Sequence
  Synthetic Polypeptide
AACAGGVLFDRCSVD

SEQ ID NO: 225 - protein, 15 aa, Artificial Sequence
  Synthetic Polypeptide
NMPACQGGSWCRPGY

SEQ ID NO: 226 - protein, 15 aa, Artificial Sequence
  Synthetic Polypeptide
TLCARPPSYQLCSHV

SEQ ID NO: 227 - protein, 15 aa, Artificial Sequence
  Synthetic Polypeptide
NLCPPGETRTQCQIT

SEQ ID NO: 228 - protein, 15 aa, Artificial Sequence
  Synthetic Polypeptide
LYCALYSVQLFCVDL

SEQ ID NO: 229 - protein, 15 aa, Artificial Sequence
  Synthetic Polypeptide
KMAPCDAWYCHQQTA

SEQ ID NO: 230 - protein, 15 aa, Artificial Sequence
  Synthetic Polypeptide
QDECSNKEAENCSDV

SEQ ID NO: 231 - protein, 15 aa, Artificial Sequence
  Synthetic Polypeptide
QTCYGWSWSGSCLWY

SEQ ID NO: 232 - protein, 15 aa, Artificial Sequence
  Synthetic Polypeptide
SNPCISTGHTHCQKI

SEQ ID NO: 233 - protein, 15 aa, Artificial Sequence
  Synthetic Polypeptide
QICFGGSKNRYDCFM

SEQ ID NO: 234 - protein, 15 aa, Artificial Sequence
  Synthetic Polypeptide
PTAPCHFNPPCRNTG

SEQ ID NO: 235 - protein, 15 aa, Artificial Sequence
  Synthetic Polypeptide
VCSGSSPGHPRVCGD

SEQ ID NO: 236 - protein, 15 aa, Artificial Sequence
  Synthetic Polypeptide
LLPCPTSMPSYCFNY

SEQ ID NO: 237 - protein, 15 aa, Artificial Sequence
  Synthetic Polypeptide
RGTPCTINTCTHHFS

SEQ ID NO: 238 - protein, 15 aa, Artificial Sequence
  Synthetic Polypeptide
KNGGCKVPIPCKSWS

SEQ ID NO: 239 - protein, 15 aa, Artificial Sequence
  Synthetic Polypeptide
SRPCSYMHPYCFYNS

SEQ ID NO: 240 - protein, 15 aa, Artificial Sequence
  Synthetic Polypeptide
SHPCSYMHPYCFYNS

SEQ ID NO: 241 - protein, 15 aa, Artificial Sequence
  Synthetic Polypeptide
SLPCSYMHPYCFYNS

SEQ ID NO: 242 - protein, 13 aa, Artificial Sequence
  Synthetic Polypeptide
ISSGLLSGRSDNH

SEQ ID NO: 243 - protein, 18 aa, Artificial Sequence
  Synthetic Polypeptide
AVGLLAPPGGLSGRSDNH

SEQ ID NO: 244 - protein, 13 aa, Artificial Sequence
  Synthetic Polypeptide
ISSGLLSGRSDIH

SEQ ID NO: 245 - protein, 13 aa, Artificial Sequence
  Synthetic Polypeptide
ISSGLLSGRSDQH

SEQ ID NO: 246 - protein, 13 aa, Artificial Sequence
  Synthetic Polypeptide
ISSGLLSGRSDNP

SEQ ID NO: 247 - protein, 13 aa, Artificial Sequence
  Synthetic Polypeptide
ISSGLLSGRSANP

SEQ ID NO: 248 - protein, 13 aa, Artificial Sequence
  Synthetic Polypeptide
ISSGLLSGRSANI

SEQ ID NO: 249 - protein, 18 aa, Artificial Sequence
  Synthetic Polypeptide
AVGLLAPPGGLSGRSDIH

SEQ ID NO: 250 - protein, 18 aa, Artificial Sequence
  Synthetic Polypeptide
AVGLLAPPGGLSGRSDQH

SEQ ID NO: 251 - protein, 18 aa, Artificial Sequence
  Synthetic Polypeptide
AVGLLAPPGGLSGRSDNP

SEQ ID NO: 252 - protein, 18 aa, Artificial Sequence
  Synthetic Polypeptide
AVGLLAPPGGLSGRSANP

SEQ ID NO: 253 - protein, 18 aa, Artificial Sequence
  Synthetic Polypeptide
AVGLLAPPGGLSGRSANI

SEQ ID NO: 254 - protein, 7 aa, Artificial Sequence
  Synthetic Polypeptide
QGQSGQG

SEQ ID NO: 255 - protein, 6 aa, Artificial Sequence
  Synthetic Polypeptide
QGQSGQ

SEQ ID NO: 256 - protein, 5 aa, Artificial Sequence
  Synthetic Polypeptide
QGQSG

SEQ ID NO: 257 - protein, 4 aa, Artificial Sequence
  Synthetic Polypeptide
QGQS

SEQ ID NO: 258 - protein, 6 aa, Artificial Sequence
  Synthetic Polypeptide
GQSGQG

SEQ ID NO: 259 - protein, 5 aa, Artificial Sequence
  Synthetic Polypeptide
QSGQG

SEQ ID NO: 260 - protein, 4 aa, Artificial Sequence
  Synthetic Polypeptide
SGQG

SEQ ID NO: 261 - protein, 158 aa, Artificial Sequence
  Synthetic Polypeptide
QGQSGQGPLMTCSDYYTCKNNLGGGSSGGSISSGLLSGRSDNIGGSDIVLTQTPLSLSVTPGQPASISCRSSRSLLHSDGFTYLYWFLQKPGQSPQLLIYQTSNLASGVPDRFSSSGSGTDFTLKISRVEAEDVGVYYCAQNLELPNTFGQGTKLEIK

SEQ ID NO: 262 - protein, 158 aa, Artificial Sequence
  Synthetic Polypeptide
QGQSGQGPLMTCSDYYTCHNNLGGGSSGGSISSGLLSGRSDNIGGSDIVLTQTPLSLSVTPGQPASISCRSSRSLLHSDGFTYLYWFLQKPGQSPQLLIYQTSNLASGVPDRFSSSGSGTDFTLKISRVEAEDVGVYYCAQNLELPNTFGQGTKLEIK

SEQ ID NO: 263 - protein, 158 aa, Artificial Sequence
  Synthetic Polypeptide
QGQSGQGPLMTCSDYYTCLNNLGGGSSGGSISSGLLSGRSDNIGGSDIVLTQTPLSLSVTPGQPASISCRSSRSLLHSDGFTYLYWFLQKPGQSPQLLIYQTSNLASGVPDRFSSSGSGTDFTLKISRVEAEDVGVYYCAQNLELPNTFGQGTKLEIK

SEQ ID NO: 264 - protein, 158 aa, Artificial Sequence
  Synthetic Polypeptide
QGQSGQGPLMTCSDYYTCRNNLGGGSSGGSISSGLLSGRSDNIGGSDIVLTQTPLSLSVTPGQPASISCRSSRSLLHSDGFTYLYWFLQKPGQSPQLLIYQTSNLASGVPDRFSSSGSGTDFTLKISRVEAEDVGVYYCAQNLELPNTFGQGTKLEIK

SEQ ID NO: 265 - protein, 158 aa, Artificial Sequence
  Synthetic Polypeptide
QGQSGQGLSCTHSRYDMHCPHMGGGSSGGSISSGLLSGRSDNIGGSDIVLTQTPLSLSVTPGQPASISCRSSRSLLHSDGFTYLYWFLQKPGQSPQLLIYQTSNLASGVPDRFSSSGSGTDFTLKISRVEAEDVGVYYCAQNLELPNTFGQGTKLEIK

SEQ ID NO: 266 - protein, 158 aa, Artificial Sequence
  Synthetic Polypeptide
QGQSGQGHYCHSRTDTITHCNAGGGSSGGSISSGLLSGRSDNIGGSDIVLTQTPLSLSVTPGQPASISCRSSRSLLHSDGFTYLYWFLQKPGQSPQLLIYQTSNLASGVPDRFSSSGSGTDFTLKISRVEAEDVGVYYCAQNLELPNTFGQGTKLEIK

SEQ ID NO: 267 - protein, 158 aa, Artificial Sequence
  Synthetic Polypeptide
QGQSGQGWCPRLFDRPSMGCPTGGGSSGGSISSGLLSGRSDNIGGSDIVLTQTPLSLSVTPGQPASISCRSSRSLLHSDGFTYLYWFLQKPGQSPQLLIYQTSNLASGVPDRFSSSGSGTDFTLKISRVEAEDVGVYYCAQNLELPNTFGQGTKLEIK

SEQ ID NO: 268 - protein, 158 aa, Artificial Sequence
  Synthetic Polypeptide
QGQSGQGWWPPCQGGAWCEQRIGGGSSGGSISSGLLSGRSDNIGGSDIVLTQTPLSLSVTPGQPASISCRSSRSLLHSDGFTYLYWFLQKPGQSPQLLIYQTSNLASGVPDRFSSSGSGTDFTLKISRVEAEDVGVYYCAQNLELPNTFGQGTKLEIK

SEQ ID NO: 269 - protein, 158 aa, Artificial Sequence
  Synthetic Polypeptide
QGQSGQGKFSCTTMPHKNCMKPGGGSSGGSISSGLLSGRSDNIGGSDIVLTQTPLSLSVTPGQPASISCRSSRSLLHSDGFTYLYWFLQKPGQSPQLLIYQTSNLASGVPDRFSSSGSGTDFTLKISRVEAEDVGVYYCAQNLELPNTFGQGTKLEIK

SEQ ID NO: 270 - protein, 158 aa, Artificial Sequence
  Synthetic Polypeptide
QGQSGQGHSGCPRLFDRCSAPAGGGSSGGSISSGLLSGRSDNIGGSDIVLTQTPLSLSVTPGQPASISCRSSRSLLHSDGFTYLYWFLQKPGQSPQLLIYQTSNLASGVPDRFSSSGSGTDFTLKISRVEAEDVGVYYCAQNLELPNTFGQGTKLEIK

SEQ ID NO: 271 - protein, 158 aa, Artificial Sequence
  Synthetic Polypeptide
QGQSGQGPLMTCTKYNNCINNLGGGSSGGSISSGLLSGRSDNIGGSDIVLTQTPLSLSVTPGQPASISCRSSRSLLHSDGFTYLYWFLQKPGQSPQLLIYQTSNLASGVPDRFSSSGSGTDFTLKISRVEAEDVGVYYCAQNLELPNTFGQGTKLEIK

SEQ ID NO: 272 - protein, 158 aa, Artificial Sequence
  Synthetic Polypeptide
QGQSGQGPNYMCKLNTCTHHIAGGGSSGGSISSGLLSGRSDNIGGSDIVLTQTPLSLSVTPGQPASISCRSSRSLLHSDGFTYLYWFLQKPGQSPQLLIYQTSNLASGVPDRFSSSGSGTDFTLKISRVEAEDVGVYYCAQNLELPNTFGQGTKLEIK

SEQ ID NO: 273 - protein, 158 aa, Artificial Sequence
  Synthetic Polypeptide
QGQSGQGAACAGGVLFDRCSVDGGGSSGGSISSGLLSGRSDNIGGSDIVLTQTPLSLSVTPGQPASISCRSSRSLLHSDGFTYLYWFLQKPGQSPQLLIYQTSNLASGVPDRFSSSGSGTDFTLKISRVEAEDVGVYYCAQNLELPNTFGQGTKLEIK

SEQ ID NO: 274 - protein, 158 aa, Artificial Sequence
  Synthetic Polypeptide
QGQSGQGFICPTLYDRPHCMHTGGGSSGGSISSGLLSGRSDNIGGSDIVLTQTPLSLSVTPGQPASISCRSSRSLLHSDGFTYLYWFLQKPGQSPQLLIYQTSNLASGVPDRFSSSGSGTDFTLKISRVEAEDVGVYYCAQNLELPNTFGQGTKLEIK

SEQ ID NO: 275 - protein, 158 aa, Artificial Sequence
  Synthetic Polypeptide
QGQSGQGNMPACQGGSWCRPGYGGGSSGGSISSGLLSGRSDNIGGSDIVLTQTPLSLSVTPGQPASISCRSSRSLLHSDGFTYLYWFLQKPGQSPQLLIYQTSNLASGVPDRFSSSGSGTDFTLKISRVEAEDVGVYYCAQNLELPNTFGQGTKLEIK

SEQ ID NO: 276 - protein, 162 aa, Artificial Sequence
  Synthetic Polypeptide
QGQSGQGPLMTCSDYYTCKNNLGGGSSGGAVGLLAPPGGLSGRSDNIGGSDIVLTQTPLSLSVTPGQPASISCRSSRSLLHSDGFTYLYWFLQKPGQSPQLLIYQTSNLASGVPDRFSSSGSGTDFTLKISRVEAEDVGVYYCAQNLELPNTFGQGTKLEIK

SEQ ID NO: 277 - protein, 162 aa, Artificial Sequence
  Synthetic Polypeptide
QGQSGQGPLMTCSDYYTCHNNLGGGSSGGAVGLLAPPGGLSGRSDNIGGSDIVLTQTPLSLSVTPGQPASISCRSSRSLLHSDGFTYLYWFLQKPGQSPQLLIYQTSNLASGVPDRFSSSGSGTDFTLKISRVEAEDVGVYYCAQNLELPNTFGQGTKLEIK

SEQ ID NO: 278 - protein, 162 aa, Artificial Sequence
  Synthetic Polypeptide
QGQSGQGPLMTCSDYYTCLNNLGGGSSGGAVGLLAPPGGLSGRSDNIGGSDIVLTQTPLSLSVTPGQPASISCRSSRSLLHSDGFTYLYWFLQKPGQSPQLLIYQTSNLASGVPDRFSSSGSGTDFTLKISRVEAEDVGVYYCAQNLELPNTFGQGTKLEIK

SEQ ID NO: 279 - protein, 162 aa, Artificial Sequence
  Synthetic Polypeptide
QGQSGQGPLMTCSDYYTCRNNLGGGSSGGAVGLLAPPGGLSGRSDNIGGSDIVLTQTPLSLSVTPGQPASISCRSSRSLLHSDGFTYLYWFLQKPGQSPQLLIYQTSNLASGVPDRFSSSGSGTDFTLKISRVEAEDVGVYYCAQNLELPNTFGQGTKLEIK

SEQ ID NO: 280 - protein, 162 aa, Artificial Sequence
  Synthetic Polypeptide
QGQSGQGLSCTHSRYDMHCPHMGGGSSGGAVGLLAPPGGLSGRSDNIGGSDIVLTQTPLSLSVTPGQPASISCRSSRSLLHSDGFTYLYWFLQKPGQSPQLLIYQTSNLASGVPDRFSSSGSGTDFTLKISRVEAEDVGVYYCAQNLELPNTFGQGTKLEIK

SEQ ID NO: 281 - protein, 162 aa, Artificial Sequence
  Synthetic Polypeptide
QGQSGQGHYCHSRTDTITHCNAGGGSSGGAVGLLAPPGGLSGRSDNIGGSDIVLTQTPLSLSVTPGQPASISCRSSRSLLHSDGFTYLYWFLQKPGQSPQLLIYQTSNLASGVPDRFSSSGSGTDFTLKISRVEAEDVGVYYCAQNLELPNTFGQGTKLEIK

SEQ ID NO: 282 - protein, 162 aa, Artificial Sequence
  Synthetic Polypeptide
QGQSGQGWCPRLFDRPSMGCPTGGGSSGGAVGLLAPPGGLSGRSDNIGGSDIVLTQTPLSLSVTPGQPASISCRSSRSLLHSDGFTYLYWFLQKPGQSPQLLIYQTSNLASGVPDRFSSSGSGTDFTLKISRVEAEDVGVYYCAQNLELPNTFGQGTKLEIK

SEQ ID NO: 283 - protein, 162 aa, Artificial Sequence
  Synthetic Polypeptide
QGQSGQGWWPPCQGGAWCEQRIGGGSSGGAVGLLAPPGGLSGRSDNIGGSDIVLTQTPLSLSVTPGQPASISCRSSRSLLHSDGFTYLYWFLQKPGQSPQLLIYQTSNLASGVPDRFSSSGSGTDFTLKISRVEAEDVGVYYCAQNLELPNTFGQGTKLEIK

SEQ ID NO: 284 - protein, 162 aa, Artificial Sequence
  Synthetic Polypeptide
QGQSGQGKFSCTTMPHKNCMKPGGGSSGGAVGLLAPPGGLSGRSDNIGGSDIVLTQTPLSLSVTPGQPASISCRSSRSLLHSDGFTYLYWFLQKPGQSPQLLIYQTSNLASGVPDRFSSSGSGTDFTLKISRVEAEDVGVYYCAQNLELPNTFGQGTKLEIK

SEQ ID NO: 285 - protein, 162 aa, Artificial Sequence
  Synthetic Polypeptide
QGQSGQGHSGCPRLFDRCSAPAGGGSSGGAVGLLAPPGGLSGRSDNIGGSDIVLTQTPLSLSVTPGQPASISCRSSRSLLHSDGFTYLYWFLQKPGQSPQLLIYQTSNLASGVPDRFSSSGSGTDFTLKISRVEAEDVGVYYCAQNLELPNTFGQGTKLEIK

SEQ ID NO: 286 - protein, 162 aa, Artificial Sequence
  Synthetic Polypeptide
QGQSGQGPLMTCTKYNNCINNLGGGSSGGAVGLLAPPGGLSGRSDNIGGSDIVLTQTPLSLSVTPGQPASISCRSSRSLLHSDGFTYLYWFLQKPGQSPQLLIYQTSNLASGVPDRFSSSGSGTDFTLKISRVEAEDVGVYYCAQNLELPNTFGQGTKLEIK

SEQ ID NO: 287 - protein, 162 aa, Artificial Sequence
  Synthetic Polypeptide
QGQSGQGPNYMCKLNTCTHHIAGGGSSGGAVGLLAPPGGLSGRSDNIGGSDIVLTQTPLSLSVTPGQPASISCRSSRSLLHSDGFTYLYWFLQKPGQSPQLLIYQTSNLASGVPDRFSSSGSGTDFTLKISRVEAEDVGVYYCAQNLELPNTFGQGTKLEIK

SEQ ID NO: 288 - protein, 162 aa, Artificial Sequence
  Synthetic Polypeptide
QGQSGQGAACAGGVLFDRCSVDGGGSSGGAVGLLAPPGGLSGRSDNIGGSDIVLTQTPLSLSVTPGQPASISCRSSRSLLHSDGFTYLYWFLQKPGQSPQLLIYQTSNLASGVPDRFSSSGSGTDFTLKISRVEAEDVGVYYCAQNLELPNTFGQGTKLEIK

SEQ ID NO: 289 - protein, 162 aa, Artificial Sequence
  Synthetic Polypeptide
QGQSGQGFICPTLYDRPHCMHTGGGSSGGAVGLLAPPGGLSGRSDNIGGSDIVLTQTPLSLSVTPGQPASISCRSSRSLLHSDGFTYLYWFLQKPGQSPQLLIYQTSNLASGVPDRFSSSGSGTDFTLKISRVEAEDVGVYYCAQNLELPNTFGQGTKLEIK

SEQ ID NO: 290 - protein, 162 aa, Artificial Sequence
  Synthetic Polypeptide
QGQSGQGNMPACQGGSWCRPGYGGGSSGGAVGLLAPPGGLSGRSDNIGGSDIVLTQTPLSLSVTPGQPASISCRSSRSLLHSDGFTYLYWFLQKPGQSPQLLIYQTSNLASGVPDRFSSSGSGTDFTLKISRVEAEDVGVYYCAQNLELPNTFGQGTKLEIK

SEQ ID NO: 291 - protein, 162 aa, Artificial Sequence
  Synthetic Polypeptide
QGQSGQGSWCHSATDTILPCSNGGGSSGGAVGLLAPPGGLSGRSDNIGGSDIVLTQTPLSLSVTPGQPASISCRSSRSLLHSDGFTYLYWFLQKPGQSPQLLIYQTSNLASGVPDRFSSSGSGTDFTLKISRVEAEDVGVYYCAQNLELPNTFGQGTKLEIK

SEQ ID NO: 292 - protein, 162 aa, Artificial Sequence
  Synthetic Polypeptide
QGQSGQGSPACSDRYYQTCVLNGGGSSGGAVGLLAPPGGLSGRSDNIGGSDIVLTQTPLSLSVTPGQPASISCRSSRSLLHSDGFTYLYWFLQKPGQSPQLLIYQTSNLASGVPDRFSSSGSGTDFTLKISRVEAEDVGVYYCAQNLELPNTFGQGTKLEIK

SEQ ID NO: 293 - protein, 162 aa, Artificial Sequence
  Synthetic Polypeptide
QGQSGQGMSCVVDRFDRQCPHLGGGSSGGAVGLLAPPGGLSGRSDNIGGSDIVLTQTPLSLSVTPGQPASISCRSSRSLLHSDGFTYLYWFLQKPGQSPQLLIYQTSNLASGVPDRFSSSGSGTDFTLKISRVEAEDVGVYYCAQNLELPNTFGQGTKLEIK

SEQ ID NO: 294 - protein, 162 aa, Artificial Sequence
  Synthetic Polypeptide
QGQSGQGTTRCEHYWFTCPLSPGGGSSGGAVGLLAPPGGLSGRSDNIGGSDIVLTQTPLSLSVTPGQPASISCRSSRSLLHSDGFTYLYWFLQKPGQSPQLLIYQTSNLASGVPDRFSSSGSGTDFTLKISRVEAEDVGVYYCAQNLELPNTFGQGTKLEIK

SEQ ID NO: 295 - protein, 162 aa, Artificial Sequence
  Synthetic Polypeptide
QGQSGQGDCTGYSPSVLPACRVGGGSSGGAVGLLAPPGGLSGRSDNIGGSDIVLTQTPLSLSVTPGQPASISCRSSRSLLHSDGFTYLYWFLQKPGQSPQLLIYQTSNLASGVPDRFSSSGSGTDFTLKISRVEAEDVGVYYCAQNLELPNTFGQGTKLEIK

SEQ ID NO: 296 - protein, 162 aa, Artificial Sequence
  Synthetic Polypeptide
QGQSGQGFCSGYSPSVLPSCLMGGGSSGGAVGLLAPPGGLSGRSDNIGGSDIVLTQTPLSLSVTPGQPASISCRSSRSLLHSDGFTYLYWFLQKPGQSPQLLIYQTSNLASGVPDRFSSSGSGTDFTLKISRVEAEDVGVYYCAQNLELPNTFGQGTKLEIK

SEQ ID NO: 297 - protein, 162 aa, Artificial Sequence
  Synthetic Polypeptide
QGQSGQGSKPCSYMHPYCFYNSGGGSSGGAVGLLAPPGGLSGRSDNIGGSDIVLTQTPLSLSVTPGQPASISCRSSRSLLHSDGFTYLYWFLQKPGQSPQLLIYQTSNLASGVPDRFSSSGSGTDFTLKISRVEAEDVGVYYCAQNLELPNTFGQGTKLEIK

SEQ ID NO: 298 - protein, 162 aa, Artificial Sequence
  Synthetic Polypeptide
QGQSGQGLTRCTIAHPYCYYNYGGGSSGGAVGLLAPPGGLSGRSDNIGGSDIVLTQTPLSLSVTPGQPASISCRSSRSLLHSDGFTYLYWFLQKPGQSPQLLIYQTSNLASGVPDRFSSSGSGTDFTLKISRVEAEDVGVYYCAQNLELPNTFGQGTKLEIK

SEQ ID NO: 299 - protein, 162 aa, Artificial Sequence
  Synthetic Polypeptide
QGQSGQGPNTCMSERRICSLTYGGGSSGGAVGLLAPPGGLSGRSDNIGGSDIVLTQTPLSLSVTPGQPASISCRSSRSLLHSDGFTYLYWFLQKPGQSPQLLIYQTSNLASGVPDRFSSSGSGTDFTLKISRVEAEDVGVYYCAQNLELPNTFGQGTKLEIK

SEQ ID NO: 300 - protein, 162 aa, Artificial Sequence
  Synthetic Polypeptide
QGQSGQGPRPHCAILRQCLAATGGGSSGGAVGLLAPPGGLSGRSDNIGGSDIVLTQTPLSLSVTPGQPASISCRSSRSLLHSDGFTYLYWFLQKPGQSPQLLIYQTSNLASGVPDRFSSSGSGTDFTLKISRVEAEDVGVYYCAQNLELPNTFGQGTKLEIK

SEQ ID NO: 301 - protein, 162 aa, Artificial Sequence
  Synthetic Polypeptide
QGQSGQGSRPCSYMHPYCFYNSGGGSSGGAVGLLAPPGGLSGRSDNIGGSDIVLTQTPLSLSVTPGQPASISCRSSRSLLHSDGFTYLYWFLQKPGQSPQLLIYQTSNLASGVPDRFSSSGSGTDFTLKISRVEAEDVGVYYCAQNLELPNTFGQGTKLEIK

SEQ ID NO: 302 - protein, 162 aa, Artificial Sequence
  Synthetic Polypeptide
QGQSGQGSHPCSYMHPYCFYNSGGGSSGGAVGLLAPPGGLSGRSDNIGGSDIVLTQTPLSLSVTPGQPASISCRSSRSLLHSDGFTYLYWFLQKPGQSPQLLIYQTSNLASGVPDRFSSSGSGTDFTLKISRVEAEDVGVYYCAQNLELPNTFGQGTKLEIK

SEQ ID NO: 303 - protein, 162 aa, Artificial Sequence
  Synthetic Polypeptide
QGQSGQGSLPCSYMHPYCFYNSGGGSSGGAVGLLAPPGGLSGRSDNIGGSDIVLTQTPLSLSVTPGQPASISCRSSRSLLHSDGFTYLYWFLQKPGQSPQLLIYQTSNLASGVPDRFSSSGSGTDFTLKISRVEAEDVGVYYCAQNLELPNTFGQGTKLEIK

SEQ ID NO: 304 - protein, 216 aa, Artificial Sequence
  Synthetic Polypeptide
APELLGGPSVFLFPPKPKDTLMISRTPEVTCVVVDVSHEDPEVKFNWYVDGVEVHNAKTKPREEQYNSTYRVVSVLTVLHQDWLNGKEYKCKVSNKALPAPIEKTISKAKGQPREPQVYTLPPSRDELTKNQVSLTCLVKGFYPSDIAVEWESNGQPENNYKTTPPVLDSDGSFFLYSKLTVDKSRWQQGNVFSCSVMHEALHNHYTQKSLSLSPG

SEQ ID NO: 305 - protein, 215 aa, Artificial Sequence
  Synthetic Polypeptide
APPVAGPSVFLFPPKPKDTLMISRTPEVTCVVVDVSHEDPEVQFNWYVDGVEVHNAKTKPREEQFNSTFRVVSVLTVVHQDWLNGKEYKCKVSNKGLPAPIEKTISKTKGQPREPQVYTLPPSREEMTKNQVSLTCLVKGFYPSDIAVEWESNGQPENNYKTTPPMLDSDGSFFLYSKLTVDKSRWQQGNVFSCSVMHEALHNHYTQKSLSLSPG

SEQ ID NO: 306 - protein, 216 aa, Artificial Sequence
  Synthetic Polypeptide
APEFLGGPSVFLFPPKPKDTLMISRTPEVTCVVVDVSQEDPEVQFNWYVDGVEVHNAKTKPREEQFNSTYRVVSVLTVLHQDWLNGKEYKCKVSNKGLPSSIEKTISKAKGQPREPQVYTLPPSQEEMTKNQVSLTCLVKGFYPSDIAVEWESNGQPENNYKTTPPVLDSDGSFFLYSRLTVDKSRWQEGNVFSCSVMHEALHNHYTQKSLSLSLG

SEQ ID NO: 307 - protein, 216 aa, Artificial Sequence
  Synthetic Polypeptide
APEAAGGPSVFLFPPKPKDTLMISRTPEVTCVVVDVSHEDPEVKFNWYVDGVEVHNAKTKPREEQYNSTYRVVSVLTVLHQDWLNGKEYKCKVSNKALPAPIEKTISKAKGQPREPQVYTLPPSRDELTKNQVSLTCLVKGFYPSDIAVEWESNGQPENNYKTTPPVLDSDGSFFLYSKLTVDKSRWQQGNVFSCSVMHEALHNHYTQKSLSLSPG

SEQ ID NO: 308 - protein, 216 aa, Artificial Sequence
  Synthetic Polypeptide
APELLGGPSVFLFPPKPKDTLMISRTPEVTCVVVDVSHEDPEVKFNWYVDGVEVHNAKTKPREEQYASTYRVVSVLTVLHQDWLNGKEYKCKVSNKALPAPIEKTISKAKGQPREPQVYTLPPSRDELTKNQVSLTCLVKGFYPSDIAVEWESNGQPENNYKTTPPVLDSDGSFFLYSKLTVDKSRWQQGNVFSCSVMHEALHNHYTQKSLSLSPG

SEQ ID NO: 309 - protein, 216 aa, Artificial Sequence
  Synthetic Polypeptide
APELLGGPSVFLFPPKPKDTLMISRTPEVTCVVVDVSHEDPEVKFNWYVDGVEVHNAKTKPREEQYQSTYRVVSVLTVLHQDWLNGKEYKCKVSNKALPAPIEKTISKAKGQPREPQVYTLPPSRDELTKNQVSLTCLVKGFYPSDIAVEWESNGQPENNYKTTPPVLDSDGSFFLYSKLTVDKSRWQQGNVFSCSVMHEALHNHYTQKSLSLSPG

SEQ ID NO: 310 - protein, 100 aa, Artificial Sequence
  Synthetic Polypeptide
DIVLTQTPFSNPVTLGTSASISCRSSKSLLHSDGFTYLYWFLQKPGQSPHLLIYQTSNLASGVPDRFSSSGSGTDFTLRISRVEAEDVGVYYCAQNLELP

SEQ ID NO: 311 - protein, 100 aa, Artificial Sequence
  Synthetic Polypeptide
DIVMTQTPLSLSVTPGQPASISCKSSQSLLHSDGKTYLYWYLQKPGQSPQLLIYEVSNRFSGVPDRFSGSGSGTDFTLKISRVEAEDVGVYYCMQSIQLP

SEQ ID NO: 312 - protein, 100 aa, Artificial Sequence
  Synthetic Polypeptide
DIVMTQTPLSLSVTPGQPASISCKSSQSLLHSDGKTYLYWYLQKPGQPPQLLIYEVSNRFSGVPDRFSGSGSGTDFTLKISRVEAEDVGVYYCMQSIQLP

SEQ ID NO: 313 - protein, 100 aa, Artificial Sequence
  Synthetic Polypeptide
DIVMTQTPLSLSVTPGQPASISCKSSQSLLHSDGKTYLYWYLQKPGQSPQLLIYEVSSRFSGVPDRFSGSGSGTDFTLKISRVEAEDVGVYYCMQGIHLP

SEQ ID NO: 314 - protein, 98 aa, Artificial Sequence
  Synthetic Polypeptide
EVKLEESGPALVKPGASVRISCKASGYTFTNYYIHWVKQRPGQGLDYIGWIYPGNVYIQYNEKFKGKATLTADKSSSTAFMQLSSLTSEDSAVYFCAR

SEQ ID NO: 315 - protein, 98 aa, Artificial Sequence
  Synthetic Polypeptide
QVQLVQSGAEVKKPGASVKVSCKASGYTFTSYAMHWVRQAPGQRLEWMGWINAGNGNTKYSQKFQGRVTITRDTSASTAYMELSSLRSEDTAVYYCAR

SEQ ID NO: 316 - protein, 98 aa, Artificial Sequence
  Synthetic Polypeptide
QVQLVQSGAEVKKPGASVKVSCKASGYTFTGYYMHWVRQAPGQGLEWMGWINPNSGGTNYAQKFQGRVTMTRDTSISTAYMELSRLRSDDTAVYYCAR

SEQ ID NO: 317 - protein, 98 aa, Artificial Sequence
  Synthetic Polypeptide
QVQLVQSGAEVKKPGASVKVSCKASGYTFTGYYMHWVRQAPGQGLEWMGWINPNSGGTNYAQKFQGWVTMTRDTSISTAYMELSRLRSDDTAVYYCAR